European Patent Specification EP 3 607 065 B1, published March 15, 2023. Title: METHOD AND KIT FOR CONSTRUCTING NUCLEIC ACID LIBRARY. Applicant: MyOmicsDx, Inc WANG, QING ZHANG, MING. The sequence listing filed with the application follows.

SEQUENCE LISTING (920 sequences)

SEQ ID NO: 1 - DNA, 23 bp, Homo Sapiens
gctcatttttgttaatggtggct

SEQ ID NO: 2 - DNA, 27 bp, Homo Sapiens
gaacaatgaataaaccattttgtctca

SEQ ID NO: 3 - DNA, 20 bp, Homo Sapiens
atcatgctgacgcttctcct

SEQ ID NO: 4 - DNA, 27 bp, Homo Sapiens
tgcagatttttaaaaagtctcttttcc

SEQ ID NO: 5 - DNA, 27 bp, Homo Sapiens
agttaataaggacatggtttctgttct

SEQ ID NO: 6 - DNA, 26 bp, Homo Sapiens
aggaaactagagttcattttcctttt

SEQ ID NO: 7 - DNA, 21 bp, Homo Sapiens
tcgcaagtctgaatcacaact

SEQ ID NO: 8 - DNA, 27 bp, Homo Sapiens
tgtgcattgagagtttttatactagtg

SEQ ID NO: 9 - DNA, 21 bp, Homo Sapiens
ccaggttagctggtaagagga

SEQ ID NO: 10 - DNA, 27 bp, Homo Sapiens
aagcttttcaggataatttctgttttt

SEQ ID NO: 11 - DNA, 22 bp, Homo Sapiens
aggatgatactggttgacacaa

SEQ ID NO: 12 - DNA, 25 bp, Homo Sapiens
tcagcttttccttaaagtcacttca

SEQ ID NO: 13 - DNA, 27 bp, Homo Sapiens
caccatatattaacttctgacatttgc

SEQ ID NO: 14 - DNA, 25 bp, Homo Sapiens
gctacaaaagagctcaacaattttt

SEQ ID NO: 15 - DNA, 25 bp, Homo Sapiens
gtgattttctaaaatagcaggctct

SEQ ID NO: 16 - DNA, 22 bp, Homo Sapiens
tcaccactgagcaaatgtttga

SEQ ID NO: 17 - DNA, 25 bp, Homo Sapiens
agcagttgtgattctttctttctac

SEQ ID NO: 18 - DNA, 27 bp, Homo Sapiens
ttggaagtataatagcagttcttttct

SEQ ID NO: 19 - DNA, 25 bp, Homo Sapiens
tgacagctatgctaatagtgtttct

SEQ ID NO: 20 - DNA, 20 bp, Homo Sapiens
tgggtgcttgggtgtgtata

SEQ ID NO: 21 - DNA, 22 bp, Homo Sapiens
tctgtcttctcctctcttcctt

SEQ ID NO: 22 - DNA, 23 bp, Homo Sapiens
tggttaggagaatgagttgttgt

SEQ ID NO: 23 - DNA, 22 bp, Homo Sapiens
tgcatctgtggcattaaatggt

SEQ ID NO: 24 - DNA, 24 bp, Homo Sapiens
atggtttttatgacacagagttgt

SEQ ID NO: 25 - DNA, 27 bp, Homo Sapiens
aggatcactttatatggatcacttttt

SEQ ID NO: 26 - DNA, 20 bp, Homo Sapiens
tgtgtacatggtgccagaat

SEQ ID NO: 27 - DNA, 26 bp, Homo Sapiens
agtcaatttttctttcttctcttgca

SEQ ID NO: 28 - DNA, 19 bp, Homo Sapiens
ttggaggccactgctatgg

SEQ ID NO: 29 - DNA, 27 bp, Homo Sapiens
aaatgtattcactgtcttctctttctt

SEQ ID NO: 30 - DNA, 23 bp, Homo Sapiens
tgtgtgactctaaattgactgca

SEQ ID NO: 31 - DNA, 27 bp, Homo Sapiens
tgtgtgacatgttctaatatagtcaca

SEQ ID NO: 32 - DNA, 22 bp, Homo Sapiens
atgcaaagtacctaactccact

SEQ ID NO: 33 - DNA, 20 bp, Homo Sapiens
tgtttgtgcctcactttgca

SEQ ID NO: 34 - DNA, 21 bp, Homo Sapiens
acacgtcttggggatatcact

SEQ ID NO: 35 - DNA, 26 bp, Homo Sapiens
actggtatggaaatattacagtcctg

SEQ ID NO: 36 - DNA, 25 bp, Homo Sapiens
gccatgttttacatttgagttcaca

SEQ ID NO: 37 - DNA, 20 bp, Homo Sapiens
acaaggctgagacctgagtt

SEQ ID NO: 38 - DNA, 22 bp, Homo Sapiens
tgtcactttgttctgtttgcag

SEQ ID NO: 39 - DNA, 20 bp, Homo Sapiens
tggctgttgtcactattgca

SEQ ID NO: 40 - DNA, 22 bp, Homo Sapiens
gctgtttctcttttctccacca

SEQ ID NO: 41 - DNA, 22 bp, Homo Sapiens
actgtgtattcatgttcccctt

SEQ ID NO: 42 - DNA, 25 bp, Homo Sapiens
ggatttaactttgtttttctctgcc

SEQ ID NO: 43 - DNA, 25 bp, Homo Sapiens
agacttcgagtgtttaaatgaaaga

SEQ ID NO: 44 - DNA, 26 bp, Homo Sapiens
tcagaagttctggaaatacttcattt

SEQ ID NO: 45 - DNA, 25 bp, Homo Sapiens
atgcttcagatgttgtatgtaatgt

SEQ ID NO: 46 - DNA, 21 bp, Homo Sapiens
ctactcatgcccctcaaactt

SEQ ID NO: 47 - DNA, 24 bp, Homo Sapiens
tcttaaatgatcctcttctcccag

SEQ ID NO: 48 - DNA, 25 bp, Homo Sapiens
gcgatgtgcatatataatggaaagg

SEQ ID NO: 49 - DNA, 20 bp, Homo Sapiens
aatcctgtttgcagcgtgag

SEQ ID NO: 50 - DNA, 26 bp, Homo Sapiens
actccattcagaaagtaattttcacc

SEQ ID NO: 51 - DNA, 24 bp, Homo Sapiens
tcaggatttttcctttctctctcc

SEQ ID NO: 52 - DNA, 21 bp, Homo Sapiens
gagttctaggctactgtggct

SEQ ID NO: 53 - DNA, 23 bp, Homo Sapiens
gtgaatacactttctgctggttt

SEQ ID NO: 54 - DNA, 22 bp, Homo Sapiens
aaccaagtcagtaaggccatat

SEQ ID NO: 55 - DNA, 23 bp, Homo Sapiens
aaacccttctgtttctttcacag

SEQ ID NO: 56 - DNA, 22 bp, Homo Sapiens
tcctgtgagtgttctgtatgtt

SEQ ID NO: 57 - DNA, 20 bp, Homo Sapiens
gctgggaacatttgtcattt

SEQ ID NO: 58 - DNA, 24 bp, Homo Sapiens
tgccgtttcgagaattttattcac

SEQ ID NO: 59 - DNA, 21 bp, Homo Sapiens
tgcacactgaaattaggacgt

SEQ ID NO: 60 - DNA, 23 bp, Homo Sapiens
tttttcccccttgatccttctag

SEQ ID NO: 61 - DNA, 20 bp, Homo Sapiens
acttattgagcatgcctggt

SEQ ID NO: 62 - DNA, 20 bp, Homo Sapiens
acgcagtgctaaccaagttc

SEQ ID NO: 63 - DNA, 25 bp, Homo Sapiens
ttttatatgatctttcctggttggc

SEQ ID NO: 64 - DNA, 20 bp, Homo Sapiens
aagaatgcctgggactgagg

SEQ ID NO: 65 - DNA, 27 bp, Homo Sapiens
aaagtgtagactaatgatgtgactttt

SEQ ID NO: 66 - DNA, 24 bp, Homo Sapiens
tgtactctttttcctgttgctgtt

SEQ ID NO: 67 - DNA, 24 bp, Homo Sapiens
aagcaaacttgttctgtttttacc

SEQ ID NO: 68 - DNA, 21 bp, Homo Sapiens
tgtgtgtttctgtgggtttct

SEQ ID NO: 69 - DNA, 22 bp, Homo Sapiens
tgtttttgtccctctctcttgc

SEQ ID NO: 70 - DNA, 26 bp, Homo Sapiens
acatactttgtatcatcttattggca

SEQ ID NO: 71 - DNA, 23 bp, Homo Sapiens
tgttttcctttgtgtcattccct

SEQ ID NO: 72 - DNA, 23 bp, Homo Sapiens
ggattcagtgaggaatgctttca

SEQ ID NO: 73 - DNA, 23 bp, Homo Sapiens
acacagaatttgttaagcaacgt

SEQ ID NO: 74 - DNA, 27 bp, Homo Sapiens
tctcatcataccactattattttgcag

SEQ ID NO: 75 - DNA, 20 bp, Homo Sapiens
acacagccttctcaacctct

SEQ ID NO: 76 - DNA, 25 bp, Homo Sapiens
ctctcggtgtatttctctacttacc

SEQ ID NO: 77 - DNA, 23 bp, Homo Sapiens
tcactgtgatagccttatctgct

SEQ ID NO: 78 - DNA, 24 bp, Homo Sapiens
gttaatcttaacctgtgctttgcc

SEQ ID NO: 79 - DNA, 20 bp, Homo Sapiens
actccaacactgttgctcct

SEQ ID NO: 80 - DNA, 20 bp, Homo Sapiens
gccagagtcctttagcccta

SEQ ID NO: 81 - DNA, 23 bp, Homo Sapiens
tcctgggtttcttttcaacttgt

SEQ ID NO: 82 - DNA, 24 bp, Homo Sapiens
tcctgaagtgagatcttacatcct

SEQ ID NO: 83 - DNA, 20 bp, Homo Sapiens
gaccagaaaggctcagttcc

SEQ ID NO: 84 - DNA, 23 bp, Homo Sapiens
aaacattgatttggcttttccca

SEQ ID NO: 85 - DNA, 20 bp, Homo Sapiens
tgtctccatttcccaccaca

SEQ ID NO: 86 - DNA, 26 bp, Homo Sapiens
atttactctggattttgctttttcag

SEQ ID NO: 87 - DNA, 22 bp, Homo Sapiens
tgagatgtttttgccttcacag

SEQ ID NO: 88 - DNA, 21 bp, Homo Sapiens
tcccccttgtcttaaaccaca

SEQ ID NO: 89 - DNA, 20 bp, Homo Sapiens
ttgacgtgccattctcttgc

SEQ ID NO: 90 - DNA, 20 bp, Homo Sapiens
tttgggacgacttattgccc

SEQ ID NO: 91 - DNA, 27 bp, Homo Sapiens
agagtaacttcaatgtctttattccat

SEQ ID NO: 92 - DNA, 20 bp, Homo Sapiens
gatctccggttgggattcct

SEQ ID NO: 93 - DNA, 23 bp, Homo Sapiens
gcattttctctgttcaacaagca

SEQ ID NO: 94 - DNA, 22 bp, Homo Sapiens
gtttgtgacataagcagaacgc

SEQ ID NO: 95 - DNA, 21 bp, Homo Sapiens
tgacagccagattcgtctttg

SEQ ID NO: 96 - DNA, 22 bp, Homo Sapiens
tggaagtctgtgagttctctga

SEQ ID NO: 97 - DNA, 26 bp, Homo Sapiens
atgttcttcctttaggtatagtctca

SEQ ID NO: 98 - DNA, 20 bp, Homo Sapiens
cctgaagcagtccaggactt

SEQ ID NO: 99 - DNA, 22 bp, Homo Sapiens
agcttaagaaaagtgacgtggt

SEQ ID NO: 100 - DNA, 27 bp, Homo Sapiens
tccttgagtgtaaggcaattaataact

SEQ ID NO: 101 - DNA, 24 bp, Homo Sapiens
gtctgtggattgacttcttttcct

SEQ ID NO: 102 - DNA, 27 bp, Homo Sapiens
tgagcctcatttattttctttttctcc

SEQ ID NO: 103 - DNA, 24 bp, Homo Sapiens
tcccttatgttcttcttctctcca

SEQ ID NO: 104 - DNA, 25 bp, Homo Sapiens
gcactttaatactaacaggaacagc

SEQ ID NO: 105 - DNA, 24 bp, Homo Sapiens
tgtcctcagtctgtactaaactca

SEQ ID NO: 106 - DNA, 22 bp, Homo Sapiens
agcagatttgtatgaaagccct

SEQ ID NO: 107 - DNA, 20 bp, Homo Sapiens
accctgttacacgcttgtaa

SEQ ID NO: 108 - DNA, 23 bp, Homo Sapiens
actgaatttgttttagggcacat

SEQ ID NO: 109 - DNA, 20 bp, Homo Sapiens
caccggtgtggctctttaac

SEQ ID NO: 110 - DNA, 20 bp, Homo Sapiens
ccgttgggttttctcttcca

SEQ ID NO: 111 - DNA, 23 bp, Homo Sapiens
ttctattcttccttgctttgtgc

SEQ ID NO: 112 - DNA, 21 bp, Homo Sapiens
aggatggtcttgtgtctgtgt

SEQ ID NO: 113 - DNA, 24 bp, Homo Sapiens
agttattttcaaacggtctggttt

SEQ ID NO: 114 - DNA, 20 bp, Homo Sapiens
aaatggcccttgtcttgcag

SEQ ID NO: 115 - DNA, 21 bp, Homo Sapiens
tctcccttcctcctttgaaca

SEQ ID NO: 116 - DNA, 23 bp, Homo Sapiens
agttaaagttcggttgttttcgt

SEQ ID NO: 117 - DNA, 20 bp, Homo Sapiens
gcaaggagccaggcattttt

SEQ ID NO: 118 - DNA, 21 bp, Homo Sapiens
tccattggattccttcgcaag

SEQ ID NO: 119 - DNA, 20 bp, Homo Sapiens
ttgtcagctttttgggggtc

SEQ ID NO: 120 - DNA, 23 bp, Homo Sapiens
ggtttacgtgcatattttctggc

SEQ ID NO: 121 - DNA, 20 bp, Homo Sapiens
ggcactttccttctggttca

SEQ ID NO: 122 - DNA, 24 bp, Homo Sapiens
tggtggtgcatactttatttgtct

SEQ ID NO: 123 - DNA, 23 bp, Homo Sapiens
aagtggtttcctcagatagagca

SEQ ID NO: 124 - DNA, 20 bp, Homo Sapiens
agcgtttcagctccagactc

SEQ ID NO: 125 - DNA, 20 bp, Homo Sapiens
agcaaccatttttgtgccca

SEQ ID NO: 126 - DNA, 20 bp, Homo Sapiens
tatgtctcctcttccctgcc

SEQ ID NO: 127 - DNA, 20 bp, Homo Sapiens
gtcctgctcctgatcctgtt

SEQ ID NO: 128 - DNA, 20 bp, Homo Sapiens
cttctccctggctctgactc

SEQ ID NO: 129 - DNA, 20 bp, Homo Sapiens
atctcaatcgcctgctctcc

SEQ ID NO: 130 - DNA, 22 bp, Homo Sapiens
agaccttttcctccctcattca

SEQ ID NO: 131 - DNA, 23 bp, Homo Sapiens
acatctgggattttgcttcattg

SEQ ID NO: 132 - DNA, 24 bp, Homo Sapiens
tcagaccacggtttctatttttca

SEQ ID NO: 133 - DNA, 25 bp, Homo Sapiens
atcttctgttacattctgcttcaca

SEQ ID NO: 134 - DNA, 20 bp, Homo Sapiens
ttttcaccccgctcccctta

SEQ ID NO: 135 - DNA, 20 bp, Homo Sapiens
tccttaaggcctctgtgctt

SEQ ID NO: 136 - DNA, 22 bp, Homo Sapiens
ggtcatttgctgtgtttgttga

SEQ ID NO: 137 - DNA, 27 bp, Homo Sapiens
ccataatataaagttgttgcgttttgt

SEQ ID NO: 138 - DNA, 22 bp, Homo Sapiens
gttctgagttagctgcacattt

SEQ ID NO: 139 - DNA, 20 bp, Homo Sapiens
ttctggccttgttaatggcg

SEQ ID NO: 140 - DNA, 23 bp, Homo Sapiens
aaatcccttcctctctttctcag

SEQ ID NO: 141 - DNA, 20 bp, Homo Sapiens
tacacccctgtcctctctgt

SEQ ID NO: 142 - DNA, 20 bp, Homo Sapiens
agacctcagacaaggcatct

SEQ ID NO: 143 - DNA, 20 bp, Homo Sapiens
actttctctcctgccctcac

SEQ ID NO: 144 - DNA, 24 bp, Homo Sapiens
cacttcagttatgtacctgatggg

SEQ ID NO: 145 - DNA, 20 bp, Homo Sapiens
ttccccattccccattccaa

SEQ ID NO: 146 - DNA, 20 bp, Homo Sapiens
tgctgaacgcatttggctta

SEQ ID NO: 147 - DNA, 21 bp, Homo Sapiens
tcattgtgtcttccctcctct

SEQ ID NO: 148 - DNA, 23 bp, Homo Sapiens
tgttgacaatgttttctcccaca

SEQ ID NO: 149 - DNA, 27 bp, Homo Sapiens
acatttttaatgctcctttctttgaca

SEQ ID NO: 150 - DNA, 21 bp, Homo Sapiens
agcaaaaggagtgacattcct

SEQ ID NO: 151 - DNA, 25 bp, Homo Sapiens
tctcatcatttcactgagatatgca

SEQ ID NO: 152 - DNA, 23 bp, Homo Sapiens
tgaacttgtcacttcattggtca

SEQ ID NO: 153 - DNA, 23 bp, Homo Sapiens
aggcagcctttataaaagcaaat

SEQ ID NO: 154 - DNA, 21 bp, Homo Sapiens
acccattttccttcctggaca

SEQ ID NO: 155 - DNA, 21 bp, Homo Sapiens
aaaaatttcccctgcgcttag

SEQ ID NO: 156 - DNA, 20 bp, Homo Sapiens
agacatgatgcttcgcttga

SEQ ID NO: 157 - DNA, 20 bp, Homo Sapiens
tgcacgttgtttgtagctgt

SEQ ID NO: 158 - DNA, 22 bp, Homo Sapiens
gtttcccctggatttatgtggt

SEQ ID NO: 159 - DNA, 20 bp, Homo Sapiens
acgtgcatgtcctttttccc

SEQ ID NO: 160 - DNA, 25 bp, Homo Sapiens
tgtctctacctcctacatcttatct

SEQ ID NO: 161 - DNA, 25 bp, Homo Sapiens
ggttgtttctatttgctaatgctgt

SEQ ID NO: 162 - DNA, 25 bp, Homo Sapiens
agcacttcctgaaataatttcacct

SEQ ID NO: 163 - DNA, 20 bp, Homo Sapiens
atgggcctcactgtctgttt

SEQ ID NO: 164 - DNA, 20 bp, Homo Sapiens
gtcctcatggctctgtgact

SEQ ID NO: 165 - DNA, 20 bp, Homo Sapiens
cccacctgcattgttcatca

SEQ ID NO: 166 - DNA, 27 bp, Homo Sapiens
ggataactatgttcttccttttcatca

SEQ ID NO: 167 - DNA, 20 bp, Homo Sapiens
ctggcacacttcttcacctc

SEQ ID NO: 168 - DNA, 20 bp, Homo Sapiens
cctcagggatggtagtgaca

SEQ ID NO: 169 - DNA, 25 bp, Homo Sapiens
catccatggaatatgttcttttgca

SEQ ID NO: 170 - DNA, 20 bp, Homo Sapiens
ccttgcactcttgtggttgt

SEQ ID NO: 171 - DNA, 23 bp, Homo Sapiens
aaggtttccaattcacctttcag

SEQ ID NO: 172 - DNA, 20 bp, Homo Sapiens
ggtccccatccattcttcct

SEQ ID NO: 173 - DNA, 22 bp, Homo Sapiens
ccaatctgcttatgaccaggag

SEQ ID NO: 174 - DNA, 21 bp, Homo Sapiens
ggtgggattttgttgtttgca

SEQ ID NO: 175 - DNA, 20 bp, Homo Sapiens
tgaccaatttggcttcgtcc

SEQ ID NO: 176 - DNA, 21 bp, Homo Sapiens
tcaaagctgcttctgtcatct

SEQ ID NO: 177 - DNA, 20 bp, Homo Sapiens
ggctaatggttctcagagct

SEQ ID NO: 178 - DNA, 22 bp, Homo Sapiens
gcctttcaattcactgtcctca

SEQ ID NO: 179 - DNA, 20 bp, Homo Sapiens
tcagcagggtttttcttgct

SEQ ID NO: 180 - DNA, 20 bp, Homo Sapiens
ggttttcctctccttcccca

SEQ ID NO: 181 - DNA, 20 bp, Homo Sapiens
ccatgacactccttccacct

SEQ ID NO: 182 - DNA, 23 bp, Homo Sapiens
tgtaattcctggcttctaggttt

SEQ ID NO: 183 - DNA, 20 bp, Homo Sapiens
cgtgttcccgtttcctcttg

SEQ ID NO: 184 - DNA, 21 bp, Homo Sapiens
cctctgtgtatctccttccca

SEQ ID NO: 185 - DNA, 20 bp, Homo Sapiens
gctttctttttgctccccca

SEQ ID NO: 186 - DNA, 21 bp, Homo Sapiens
acttttaccctggatttgccc

SEQ ID NO: 187 - DNA, 21 bp, Homo Sapiens
ggtggggttttgttaacgtga

SEQ ID NO: 188 - DNA, 24 bp, Homo Sapiens
agtgtaaagttaaccttgctgtgt

SEQ ID NO: 189 - DNA, 20 bp, Homo Sapiens
gtatcaaggctgccctgact

SEQ ID NO: 190 - DNA, 20 bp, Homo Sapiens
ttcaggccaccaacctcatt

SEQ ID NO: 191 - DNA, 20 bp, Homo Sapiens
gtgctgattccctgatgtgc

SEQ ID NO: 192 - DNA, 20 bp, Homo Sapiens
accaacatggatggagtggt

SEQ ID NO: 193 - DNA, 19 bp, Homo Sapiens
tgcccaccctaatcctgtg

SEQ ID NO: 194 - DNA, 20 bp, Homo Sapiens
ctgcctctcttttctcccca

SEQ ID NO: 195 - DNA, 20 bp, Homo Sapiens
gaagtcatgggctgcttgtc

SEQ ID NO: 196 - DNA, 20 bp, Homo Sapiens
ccaagctgtgaaggcctttt

SEQ ID NO: 197 - DNA, 20 bp, Homo Sapiens
cctccttctcacgtgtctgt

SEQ ID NO: 198 - DNA, 20 bp, Homo Sapiens
agcagagtgacccagtgatg

SEQ ID NO: 199 - DNA, 20 bp, Homo Sapiens
tcctctctggatcctcgtga

SEQ ID NO: 200 - DNA, 20 bp, Homo Sapiens
ggagctgctcctcatcctac

SEQ ID NO: 201 - DNA, 23 bp, Homo Sapiens
tgaagtttttgtctgtttctccc

SEQ ID NO: 202 - DNA, 20 bp, Homo Sapiens
actggatctgcttcacacct

SEQ ID NO: 203 - DNA, 20 bp, Homo Sapiens
ctttccctcattccctcccc

SEQ ID NO: 204 - DNA, 20 bp, Homo Sapiens
ttgggcctgtgttatctcct

SEQ ID NO: 205 - DNA, 20 bp, Homo Sapiens
cctgacccttctccctatcc

SEQ ID NO: 206 - DNA, 20 bp, Homo Sapiens
tccctttctcccctctttga

SEQ ID NO: 207 - DNA, 20 bp, Homo Sapiens
actcaagtccctttcccctc

SEQ ID NO: 208 - DNA, 20 bp, Homo Sapiens
tcttcacttcagttgcccct

SEQ ID NO: 209 - DNA, 20 bp, Homo Sapiens
ccacactgagcctttttccc

SEQ ID NO: 210 - DNA, 19 bp, Homo Sapiens
catgatgcgctgtgtgtcc

SEQ ID NO: 211 - DNA, 20 bp, Homo Sapiens
aggaagggcagtgaggattc

SEQ ID NO: 212 - DNA, 20 bp, Homo Sapiens
caaaaagtgccagccctcac

SEQ ID NO: 213 - DNA, 20 bp, Homo Sapiens
actaagttgccacaggacct

SEQ ID NO: 214 - DNA, 20 bp, Homo Sapiens
gggctctggggcattaacat

SEQ ID NO: 215 - DNA, 20 bp, Homo Sapiens
cgaagtctcgctcttttccc

SEQ ID NO: 216 - DNA, 25 bp, Homo Sapiens
tgttttgttgttcttggcattttct

SEQ ID NO: 217 - DNA, 20 bp, Homo Sapiens
acctgcccagatccttaacc

SEQ ID NO: 218 - DNA, 20 bp, Homo Sapiens
ctctctccacccaaaccctt

SEQ ID NO: 219 - DNA, 21 bp, Homo Sapiens
tcccctcctcttcttgttctc

SEQ ID NO: 220 - DNA, 21 bp, Homo Sapiens
cgacttcagtcttccacttcc

SEQ ID NO: 221 - DNA, 20 bp, Homo Sapiens
tcagcaggaagtgttgacct

SEQ ID NO: 222 - DNA, 20 bp, Homo Sapiens
gaggccaggcatttttcact

SEQ ID NO: 223 - DNA, 20 bp, Homo Sapiens
caacacagtctctccctcca

SEQ ID NO: 224 - DNA, 19 bp, Homo Sapiens
ttgctgctgcctcgcttat

SEQ ID NO: 225 - DNA, 20 bp, Homo Sapiens
actgttctgacacaccccac

SEQ ID NO: 226 - DNA, 20 bp, Homo Sapiens
ctctaaatccctcgccctgg

SEQ ID NO: 227 - DNA, 20 bp, Homo Sapiens
aacctctacccacccattcc

SEQ ID NO: 228 - DNA, 20 bp, Homo Sapiens
tcctctctccccactctcag

SEQ ID NO: 229 - DNA, 18 bp, Homo Sapiens
aaaaacgggtggttgggc

SEQ ID NO: 230 - DNA, 20 bp, Homo Sapiens
acagacagccgaacagacac

SEQ ID NO: 231 - DNA, 25 bp, Homo Sapiens
ttctttttagtctagtgctccacta

SEQ ID NO: 232 - DNA, 19 bp, Homo Sapiens
taagcccgggacttccttg

SEQ ID NO: 233 - DNA, 20 bp, Homo Sapiens
ggggttttgattggctgagg

SEQ ID NO: 234 - DNA, 20 bp, Homo Sapiens
cctagggtgaggcttatggg

SEQ ID NO: 235 - DNA, 20 bp, Homo Sapiens
gggtggccattaacacacaa

SEQ ID NO: 236 - DNA, 20 bp, Homo Sapiens
ctgcgaggaggggagaattc

SEQ ID NO: 237 - DNA, 20 bp, Homo Sapiens
tcccattcccgtgtttcctt

SEQ ID NO: 238 - DNA, 20 bp, Homo Sapiens
aggctctgatgtgcttctct

SEQ ID NO: 239 - DNA, 20 bp, Homo Sapiens
gttttctgtctgcctctgcc

SEQ ID NO: 240 - DNA, 20 bp, Homo Sapiens
accctcaccctaaatctggc

SEQ ID NO: 241 - DNA, 19 bp, Homo Sapiens
ctgagcctgccctactctg

SEQ ID NO: 242 - DNA, 18 bp, Homo Sapiens
cgcgcgtacacacacaca

SEQ ID NO: 243 - DNA, 20 bp, Homo Sapiens
cctctctccttctgcctcag

SEQ ID NO: 244 - DNA, 22 bp, Homo Sapiens
tcgctgttagacatctctctca

SEQ ID NO: 245 - DNA, 20 bp, Homo Sapiens
tgagaccccttcagacccta

SEQ ID NO: 246 - DNA, 20 bp, Homo Sapiens
gtgtttccttggggtcatgg

SEQ ID NO: 247 - DNA, 18 bp, Homo Sapiens
ctcgctcatccccgaggg

SEQ ID NO: 248 - DNA, 20 bp, Homo Sapiens
ggcagctccgggtctataaa

SEQ ID NO: 249 - DNA, 20 bp, Homo Sapiens
ccctcaccttcccctctttt

SEQ ID NO: 250 - DNA, 20 bp, Homo Sapiens
ctgtccttccctgacctcag

SEQ ID NO: 251 - DNA, 18 bp, Homo Sapiens
tggtctctcggcgggaag

SEQ ID NO: 252 - DNA, 20 bp, Homo Sapiens
tgagttaacggctgcctctt

SEQ ID NO: 253 - DNA, 20 bp, Homo Sapiens
cacctggctccactgtgtag

SEQ ID NO: 254 - DNA, 20 bp, Homo Sapiens
cccctgctaatgtctgaggt

SEQ ID NO: 255 - DNA, 18 bp, Homo Sapiens
ctggccacactgggtctc

SEQ ID NO: 256 - DNA, 20 bp, Homo Sapiens
cactgtggccttgtttcctg

SEQ ID NO: 257 - DNA, 18 bp, Homo Sapiens
ctcactcctcccctgctc

SEQ ID NO: 258 - DNA, 20 bp, Homo Sapiens
tagttggcgagtgggcttta

SEQ ID NO: 259 - DNA, 19 bp, Homo Sapiens
ctggtttagcgacacgagc

SEQ ID NO: 260 - DNA, 20 bp, Homo Sapiens
cctctgctgactctgtctcc

SEQ ID NO: 261 - DNA, 19 bp, Homo Sapiens
cattggttgcggccatctc

SEQ ID NO: 262 - DNA, 18 bp, Homo Sapiens
ccactgcaacccgactcc

SEQ ID NO: 263 - DNA, 18 bp, Homo Sapiens
caggagggcggggtaaag

SEQ ID NO: 264 - DNA, 18 bp, Homo Sapiens
cgcctcttcccaccctag

SEQ ID NO: 265 - DNA, 18 bp, Homo Sapiens
cgtgaccgacatgtggct

SEQ ID NO: 266 - DNA, 20 bp, Homo Sapiens
ctgagacctggggactgatc

SEQ ID NO: 267 - DNA, 20 bp, Homo Sapiens
agggtttccttctcgctgat

SEQ ID NO: 268 - DNA, 18 bp, Homo Sapiens
aggtgtggtgttgcccac

SEQ ID NO: 269 - DNA, 20 bp, Homo Sapiens
tacccactccatttcccacc

SEQ ID NO: 270 - DNA, 18 bp, Homo Sapiens
ctgggctggcgtatgacg

SEQ ID NO: 271 - DNA, 20 bp, Homo Sapiens
ccgctcagtgtctctctctt

SEQ ID NO: 272 - DNA, 19 bp, Homo Sapiens
caggaagcctgtgttccgt

SEQ ID NO: 273 - DNA, 20 bp, Homo Sapiens
gaacttgccggttaagcagg

SEQ ID NO: 274 - DNA, 20 bp, Homo Sapiens
gtatcaacgctctgtgggtc

SEQ ID NO: 275 - DNA, 20 bp, Homo Sapiens
tgcttctcttccttctcccc

SEQ ID NO: 276 - DNA, 18 bp, Homo Sapiens
ctttgtgtgccccgctcc

SEQ ID NO: 277 - DNA, 19 bp, Homo Sapiens
aggcctcttgtttcctccc

SEQ ID NO: 278 - DNA, 20 bp, Homo Sapiens
ctatgggtgcccttctccac

SEQ ID NO: 279 - DNA, 19 bp, Homo Sapiens
gaggacctgtgggactctg

SEQ ID NO: 280 - DNA, 20 bp, Homo Sapiens
gggtgagactgacctctctt

SEQ ID NO: 281 - DNA, 18 bp, Homo Sapiens
ctgcagttcgcttgtgcc

SEQ ID NO: 282 - DNA, 18 bp, Homo Sapiens
cacccaccgctgtgttgc

SEQ ID NO: 283 - DNA, 19 bp, Homo Sapiens
aggaagggagcctcaaagg

SEQ ID NO: 284 - DNA, 19 bp, Homo Sapiens
gactctcctgtctccgctc

SEQ ID NO: 285 - DNA, 18 bp, Homo Sapiens
cctcctctgcgttcgacg

SEQ ID NO: 286 - DNA, 20 bp, Homo Sapiens
actacatttcccaggaggca

SEQ ID NO: 287 - DNA, 18 bp, Homo Sapiens
ccgtccgcgctacatact

SEQ ID NO: 288 - DNA, 20 bp, Homo Sapiens
cagtggctcaggaaaccaag

SEQ ID NO: 289 - DNA, 20 bp, Homo Sapiens
gctgatcctccaccttcctt

SEQ ID NO: 290 - DNA, 19 bp, Homo Sapiens
gaacatggtgcgcaggttc

SEQ ID NO: 291 - DNA, 20 bp, Homo Sapiens
gtgtgttgggggatagcctc

SEQ ID NO: 292 - DNA, 18 bp, Homo Sapiens
cacgtctgcccctctctc

SEQ ID NO: 293 - DNA, 19 bp, Homo Sapiens
ggcagaagagaggcagaca

SEQ ID NO: 294 - DNA, 20 bp, Homo Sapiens
tattaccggcagaaccagca

SEQ ID NO: 295 - DNA, 20 bp, Homo Sapiens
cacccggttccatctacctt

SEQ ID NO: 296 - DNA, 18 bp, Homo Sapiens
cgatgagggtctggccag

SEQ ID NO: 297 - DNA, 18 bp, Homo Sapiens
cgctgctgccttgatggg

SEQ ID NO: 298 - DNA, 20 bp, Homo Sapiens
actcactgaccctctccctt

SEQ ID NO: 299 - DNA, 20 bp, Homo Sapiens
agcgaggacatctggaagaa

SEQ ID NO: 300 - DNA, 19 bp, Homo Sapiens
caagaggccaatgaggggg

SEQ ID NO: 301 - DNA, 20 bp, Homo Sapiens
ctacctgtaactgggcctgt

SEQ ID NO: 302 - DNA, 18 bp, Homo Sapiens
gatggcgcctcagaagca

SEQ ID NO: 303 - DNA, 18 bp, Homo Sapiens
gggctccgtagacgcttt

SEQ ID NO: 304 - DNA, 20 bp, Homo Sapiens
ctgccttctcccctgaagag

SEQ ID NO: 305 - DNA, 27 bp, Homo Sapiens
agttgttttagaagatatttgcaagca

SEQ ID NO: 306 - DNA, 27 bp, Homo Sapiens
tcttatcttcactgaaaacataaacct

SEQ ID NO: 307 - DNA, 25 bp, Homo Sapiens
actgaaagctaggcacattttatga

SEQ ID NO: 308 - DNA, 23 bp, Homo Sapiens
gggggaaaagaacatctgaaaat

SEQ ID NO: 309 - DNA, 26 bp, Homo Sapiens
tgagaatacatttccaaacttgtcct

SEQ ID NO: 310 - DNA, 25 bp, Homo Sapiens
acattagcaattaagaacaccatct

SEQ ID NO: 311 - DNA, 23 bp, Homo Sapiens
tggtaaaacacaatccttcacga

SEQ ID NO: 312 - DNA, 24 bp, Homo Sapiens
acctgtagttcaactaaacagagg

SEQ ID NO: 313 - DNA, 20 bp, Homo Sapiens
acgcaactgacaggaggaat

SEQ ID NO: 314 - DNA, 23 bp, Homo Sapiens
tgccttatttccctattgatgca

SEQ ID NO: 315 - DNA, 25 bp, Homo Sapiens
tcactaaatacgtttcacaggtaga

SEQ ID NO: 316 - DNA, 25 bp, Homo Sapiens
tcagaaacgatcagttgaaatttca

SEQ ID NO: 317 - DNA, 27 bp, Homo Sapiens
tgcataagttatcaaaacacttaaggt

SEQ ID NO: 318 - DNA, 23 bp, Homo Sapiens
tttatgctctcccaataagctcc

SEQ ID NO: 319 - DNA, 19 bp, Homo Sapiens
gcgcccggctgaaattttt

SEQ ID NO: 320 - DNA, 24 bp, Homo Sapiens
ctcaaaggtacatgagaaaggtga

SEQ ID NO: 321 - DNA, 25 bp, Homo Sapiens
acaatagtacggtaatgaagaagct

SEQ ID NO: 322 - DNA, 24 bp, Homo Sapiens
atggctacatgtaactagtgagat

SEQ ID NO: 323 - DNA, 27 bp, Homo Sapiens
tcctagtcctttaaaacttttacgtga

SEQ ID NO: 324 - DNA, 22 bp, Homo Sapiens
actttcaaccactctgaaaggt

SEQ ID NO: 325 - DNA, 23 bp, Homo Sapiens
actttgcactgaaaaagtacaca

SEQ ID NO: 326 - DNA, 20 bp, Homo Sapiens
gacagctccttcaagaggga

SEQ ID NO: 327 - DNA, 21 bp, Homo Sapiens
catacaggttgccttactggt

SEQ ID NO: 328 - DNA, 26 bp, Homo Sapiens
agtttaaaatcatatgcacaacctca

SEQ ID NO: 329 - DNA, 25 bp, Homo Sapiens
gcgggtgatacttctttaatactca

SEQ ID NO: 330 - DNA, 20 bp, Homo Sapiens
tgcacccccataaatccaaa

SEQ ID NO: 331 - DNA, 22 bp, Homo Sapiens
acagacagaaattcactctgca

SEQ ID NO: 332 - DNA, 25 bp, Homo Sapiens
aacaaaccttatttcccacatgtaa

SEQ ID NO: 333 - DNA, 24 bp, Homo Sapiens
tcaataatgcatttccactccaaa

SEQ ID NO: 334 - DNA, 24 bp, Homo Sapiens
tgaagtgatcggaatacatgtaga

SEQ ID NO: 335 - DNA, 21 bp, Homo Sapiens
ggtcctgcaccagtaatatgc

SEQ ID NO: 336 - DNA, 20 bp, Homo Sapiens
gcctatgtgacagcaaacca

SEQ ID NO: 337 - DNA, 22 bp, Homo Sapiens
tcagtggcatcttttcacaagt

SEQ ID NO: 338 - DNA, 23 bp, Homo Sapiens
tcaggggtatctcacatactagc

SEQ ID NO: 339 - DNA, 21 bp, Homo Sapiens
ggaacaaagaaaaggccagga

SEQ ID NO: 340 - DNA, 25 bp, Homo Sapiens
tctatggtaaaagatctcaggtcat

SEQ ID NO: 341 - DNA, 25 bp, Homo Sapiens
tcaaggaaagctgatacctatttca

SEQ ID NO: 342 - DNA, 20 bp, Homo Sapiens
ttccaacctccaatgaccca

SEQ ID NO: 343 - DNA, 24 bp, Homo Sapiens
tgtccttgtgaaataaaaagaccc

SEQ ID NO: 344 - DNA, 24 bp, Homo Sapiens
aaacccactaatacttgaaggtca

SEQ ID NO: 345 - DNA, 20 bp, Homo Sapiens
cccacttccaaactcaagcc

SEQ ID NO: 346 - DNA, 24 bp, Homo Sapiens
aacaaaaacctgagaaaccagaac

SEQ ID NO: 347 - DNA, 20 bp, Homo Sapiens
taaattgcaaagcccacccc

SEQ ID NO: 348 - DNA, 21 bp, Homo Sapiens
tgaggggaacatatgtgcaac

SEQ ID NO: 349 - DNA, 23 bp, Homo Sapiens
acgtttacatactgaacacaggt

SEQ ID NO: 350 - DNA, 21 bp, Homo Sapiens
ccgagcagtcaaatgaactca

SEQ ID NO: 351 - DNA, 23 bp, Homo Sapiens
acagcaatcgtgaacaaatacct

SEQ ID NO: 352 - DNA, 27 bp, Homo Sapiens
ttttcattcgtatatgcttttcaaaca

SEQ ID NO: 353 - DNA, 22 bp, Homo Sapiens
tgaaacctgagaagaaggatgt

SEQ ID NO: 354 - DNA, 20 bp, Homo Sapiens
aggacttcactgtgacctgg

SEQ ID NO: 355 - DNA, 20 bp, Homo Sapiens
tgcttcaatggaggagctca

SEQ ID NO: 356 - DNA, 22 bp, Homo Sapiens
ggaccaagacatcacattccag

SEQ ID NO: 357 - DNA, 20 bp, Homo Sapiens
aatgtgggatcctcgcctta

SEQ ID NO: 358 - DNA, 27 bp, Homo Sapiens
cagtataattaacccaatattcggagt

SEQ ID NO: 359 - DNA, 20 bp, Homo Sapiens
tgtgttattggcaggaacgt

SEQ ID NO: 360 - DNA, 22 bp, Homo Sapiens
agaaagtacagaagaaggggga

SEQ ID NO: 361 - DNA, 23 bp, Homo Sapiens
tgtactgaaatgccaatggaact

SEQ ID NO: 362 - DNA, 21 bp, Homo Sapiens
tgtcccttcaacatcaaccaa

SEQ ID NO: 363 - DNA, 22 bp, Homo Sapiens
tgaaaccctcatgttaagcaac

SEQ ID NO: 364 - DNA, 18 bp, Homo Sapiens
aagccgtccgagatgacc

SEQ ID NO: 365 - DNA, 20 bp, Homo Sapiens
ggccaatctgctctaaacca

SEQ ID NO: 366 - DNA, 24 bp, Homo Sapiens
tgcaaaccacaaaagtatactcca

SEQ ID NO: 367 - DNA, 22 bp, Homo Sapiens
acaaagcacgatatgaagcaca

SEQ ID NO: 368 - DNA, 23 bp, Homo Sapiens
tcctaaacgtaagaagcaacact

SEQ ID NO: 369 - DNA, 23 bp, Homo Sapiens
tatgtaagacacgagacactgga

SEQ ID NO: 370 - DNA, 24 bp, Homo Sapiens
tcacaaccattaaaacaggagaca

SEQ ID NO: 371 - DNA, 25 bp, Homo Sapiens
agacaacgtcttcctatgatagaaa

SEQ ID NO: 372 - DNA, 23 bp, Homo Sapiens
cccaagatttaagaccaaaggct

SEQ ID NO: 373 - DNA, 27 bp, Homo Sapiens
tcaaaatagaatttagttgatggaggg

SEQ ID NO: 374 - DNA, 20 bp, Homo Sapiens
gcaatcccaggccagagata

SEQ ID NO: 375 - DNA, 27 bp, Homo Sapiens
tggagtttttctattaaccaggttatt

SEQ ID NO: 376 - DNA, 21 bp, Homo Sapiens
tgcagatatggcatcaacaga

SEQ ID NO: 377 - DNA, 20 bp, Homo Sapiens
ctccaaacctctacctggca

SEQ ID NO: 378 - DNA, 20 bp, Homo Sapiens
tgtgcagtccaggaaacaga

SEQ ID NO: 379 - DNA, 23 bp, Homo Sapiens
ttatgctgcttatcatacccagt

SEQ ID NO: 380 - DNA, 22 bp, Homo Sapiens
tcatgtccccagaaaatccagt

SEQ ID NO: 381 - DNA, 24 bp, Homo Sapiens
ctgactctagatacctggctaaac

SEQ ID NO: 382 - DNA, 27 bp, Homo Sapiens
aaaaaggcaccatctaaaagaaatagt

SEQ ID NO: 383 - DNA, 22 bp, Homo Sapiens
cttggagcaagtaagagcatgt

SEQ ID NO: 384 - DNA, 22 bp, Homo Sapiens
cgcagacaaatttcaggaagga

SEQ ID NO: 385 - DNA, 23 bp, Homo Sapiens
gcctacttcatccaaaatagcca

SEQ ID NO: 386 - DNA, 27 bp, Homo Sapiens
tctctaacacgactataattttcctct

SEQ ID NO: 387 - DNA, 24 bp, Homo Sapiens
tcaagagataaagtccataagcct

SEQ ID NO: 388 - DNA, 19 bp, Homo Sapiens
cccatttggaagcagctcg

SEQ ID NO: 389 - DNA, 20 bp, Homo Sapiens
tggctaaccaagtctcagga

SEQ ID NO: 390 - DNA, 25 bp, Homo Sapiens
ccagttatatcacaaataaagcccc

SEQ ID NO: 391 - DNA, 20 bp, Homo Sapiens
atctgaagatggggctggtg

SEQ ID NO: 392 - DNA, 24 bp, Homo Sapiens
aacattgcatattacccacaaaga

SEQ ID NO: 393 - DNA, 25 bp, Homo Sapiens
acaacaggaagtaaactcattttcc

SEQ ID NO: 394 - DNA, 20 bp, Homo Sapiens
agaattcaggcaatcaccca

SEQ ID NO: 395 - DNA, 21 bp, Homo Sapiens
agggtgtttctgtaacctcca

SEQ ID NO: 396 - DNA, 20 bp, Homo Sapiens
accaatttcctgtgcagaga

SEQ ID NO: 397 - DNA, 20 bp, Homo Sapiens
acagaaagctcccactcctc

SEQ ID NO: 398 - DNA, 25 bp, Homo Sapiens
agacaattcaagcttcagaatctct

SEQ ID NO: 399 - DNA, 24 bp, Homo Sapiens
ctcctctcagtcttctaaaatggt

SEQ ID NO: 400 - DNA, 21 bp, Homo Sapiens
tggaagggtttatatcgggct

SEQ ID NO: 401 - DNA, 23 bp, Homo Sapiens
tctgaaccacaatcaacttctcc

SEQ ID NO: 402 - DNA, 21 bp, Homo Sapiens
aacactgtgaaaagcaaagct

SEQ ID NO: 403 - DNA, 22 bp, Homo Sapiens
tctactgccaatgccttagttc

SEQ ID NO: 404 - DNA, 20 bp, Homo Sapiens
gtggcaaggttgaatcagca

SEQ ID NO: 405 - DNA, 25 bp, Homo Sapiens
tgctttaaaatctactcctaccagg

SEQ ID NO: 406 - DNA, 21 bp, Homo Sapiens
tggagccacataacacattca

SEQ ID NO: 407 - DNA, 22 bp, Homo Sapiens
agagaatgatgcaatttggggt

SEQ ID NO: 408 - DNA, 21 bp, Homo Sapiens
tttgcagccagaatctcttcc

SEQ ID NO: 409 - DNA, 24 bp, Homo Sapiens
agagaacagagaaagcttgaaact

SEQ ID NO: 410 - DNA, 20 bp, Homo Sapiens
cactgagagccttgaaagcc

SEQ ID NO: 411 - DNA, 22 bp, Homo Sapiens
ggaaacatcctgcacgttaagt

SEQ ID NO: 412 - DNA, 20 bp, Homo Sapiens
acactgacattgggagttgg

SEQ ID NO: 413 - DNA, 25 bp, Homo Sapiens
tgtacttaccacaacaaccttatct

SEQ ID NO: 414 - DNA, 20 bp, Homo Sapiens
gggccttgcagtaaaaggag

SEQ ID NO: 415 - DNA, 23 bp, Homo Sapiens
gcttgatctggagttaatcgaga

SEQ ID NO: 416 - DNA, 20 bp, Homo Sapiens
gtgggttttagcttgtcgca

SEQ ID NO: 417 - DNA, 20 bp, Homo Sapiens
ctggctccagaatccttcct

SEQ ID NO: 418 - DNA, 20 bp, Homo Sapiens
aagggggattctatgcctgg

SEQ ID NO: 419 - DNA, 21 bp, Homo Sapiens
agcatcctcccaaaagaagga

SEQ ID NO: 420 - DNA, 24 bp, Homo Sapiens
aatacagtaaggagtggagaagtc

SEQ ID NO: 421 - DNA, 23 bp, Homo Sapiens
cctgacaaatccagagtatacgc

SEQ ID NO: 422 - DNA, 24 bp, Homo Sapiens
agacccattaaaacctattcctca

SEQ ID NO: 423 - DNA, 21 bp, Homo Sapiens
ggcaaaagcctttgatgaagc

SEQ ID NO: 424 - DNA, 20 bp, Homo Sapiens
gtggaataacacctccagcc

SEQ ID NO: 425 - DNA, 25 bp, Homo Sapiens
tgatttttaaagtagcagaatggca

SEQ ID NO: 426 - DNA, 21 bp, Homo Sapiens
tgagtcacacaccaatgaaga

SEQ ID NO: 427 - DNA, 23 bp, Homo Sapiens
gtgaaatatgcaacagcttctca

SEQ ID NO: 428 - DNA, 23 bp, Homo Sapiens
tttacacggaatttcagtggtgg

SEQ ID NO: 429 - DNA, 21 bp, Homo Sapiens
acgaatcacttcttcagggga

SEQ ID NO: 430 - DNA, 20 bp, Homo Sapiens
aaggaaagccccttgagttt

SEQ ID NO: 431 - DNA, 25 bp, Homo Sapiens
acaacccacagtattttaaattgca

SEQ ID NO: 432 - DNA, 21 bp, Homo Sapiens
ccccagtaagtcccttcaaat

SEQ ID NO: 433 - DNA, 24 bp, Homo Sapiens
accacatatctgctatgtcttcct

SEQ ID NO: 434 - DNA, 24 bp, Homo Sapiens
tgactgaatgagaacttaagtggg

SEQ ID NO: 435 - DNA, 21 bp, Homo Sapiens
ccctcccatcttcctctaacc

SEQ ID NO: 436 - DNA, 20 bp, Homo Sapiens
acactggcatgcaacatgtt

SEQ ID NO: 437 - DNA, 20 bp, Homo Sapiens
aaacaggcctgagaaagctt

SEQ ID NO: 438 - DNA, 19 bp, Homo Sapiens
atccgtgatctgcaggcat

SEQ ID NO: 439 - DNA, 19 bp, Homo Sapiens
ccacacctggccaagctta

SEQ ID NO: 440 - DNA, 23 bp, Homo Sapiens
tctgtcatcacactcaaagatgc

SEQ ID NO: 441 - DNA, 18 bp, Homo Sapiens
tctgacacgcaagcccag

SEQ ID NO: 442 - DNA, 19 bp, Homo Sapiens
gcgcagaaagtgacagtgc

SEQ ID NO: 443 - DNA, 21 bp, Homo Sapiens
ccccctcgattgttaacatga

SEQ ID NO: 444 - DNA, 20 bp, Homo Sapiens
tcatgaacttcccacacagc

SEQ ID NO: 445 - DNA, 20 bp, Homo Sapiens
tcccaacaccggaaaggata

SEQ ID NO: 446 - DNA, 20 bp, Homo Sapiens
catcccagccatacaggact

SEQ ID NO: 447 - DNA, 20 bp, Homo Sapiens
ctatgctgcagctgttaccc

SEQ ID NO: 448 - DNA, 20 bp, Homo Sapiens
tggaaggcagtaaaggctga

SEQ ID NO: 449 - DNA, 20 bp, Homo Sapiens
acactctgacaggtcaagca

SEQ ID NO: 450 - DNA, 20 bp, Homo Sapiens
taaaccctaccccaagcagc

SEQ ID NO: 451 - DNA, 21 bp, Homo Sapiens
actcaaggcataaaagctggg

SEQ ID NO: 452 - DNA, 20 bp, Homo Sapiens
cctgacaaagtgcaggactc

SEQ ID NO: 453 - DNA, 21 bp, Homo Sapiens
gtgattttcgtggaagtgggt

SEQ ID NO: 454 - DNA, 20 bp, Homo Sapiens
tccaagctagtagtggccag

SEQ ID NO: 455 - DNA, 20 bp, Homo Sapiens
ggtcacacatgggtctgagg

SEQ ID NO: 456 - DNA, 19 bp, Homo Sapiens
caggccacacacacacttc

SEQ ID NO: 457 - DNA, 24 bp, Homo Sapiens
atagcccttacaacaaaaacaaga

SEQ ID NO: 458 - DNA, 20 bp, Homo Sapiens
gccagagcaggattaggaga

SEQ ID NO: 459 - DNA, 20 bp, Homo Sapiens
cagtgcgtgctcctttagtg

SEQ ID NO: 460 - DNA, 22 bp, Homo Sapiens
gctctgaaaatgctctttggga

SEQ ID NO: 461 - DNA, 26 bp, Homo Sapiens
tggacatttgtagaagaaataaggct

SEQ ID NO: 462 - DNA, 20 bp, Homo Sapiens
caccttcgcctttactgcag

SEQ ID NO: 463 - DNA, 22 bp, Homo Sapiens
attccttgaccacatcaaacct

SEQ ID NO: 464 - DNA, 20 bp, Homo Sapiens
agcacctcctactccctact

SEQ ID NO: 465 - DNA, 21 bp, Homo Sapiens
gacacccaaacaaggaactca

SEQ ID NO: 466 - DNA, 20 bp, Homo Sapiens
gagaccctctcttcagagcc

SEQ ID NO: 467 - DNA, 20 bp, Homo Sapiens
caatgatgctggtccacacc

SEQ ID NO: 468 - DNA, 21 bp, Homo Sapiens
aggagcttcatgacagactca

SEQ ID NO: 469 - DNA, 21 bp, Homo Sapiens
tgcagggcttcatacaagaga

SEQ ID NO: 470 - DNA, 19 bp, Homo Sapiens
ctcctcttctctggcagcc

SEQ ID NO: 471 - DNA, 20 bp, Homo Sapiens
ctgctcccctgtgaatcagt

SEQ ID NO: 472 - DNA, 20 bp, Homo Sapiens
agatcctgcacttgctcact

SEQ ID NO: 473 - DNA, 19 bp, Homo Sapiens
tccctccatgctcctctct

SEQ ID NO: 474 - DNA, 20 bp, Homo Sapiens
caaatatcagggtgcagggc

SEQ ID NO: 475 - DNA, 20 bp, Homo Sapiens
gattcatttctgctgggccc

SEQ ID NO: 476 - DNA, 20 bp, Homo Sapiens
ggtagtccagggtatgtggg

SEQ ID NO: 477 - DNA, 22 bp, Homo Sapiens
cacttatgcaaggagaatgctg

SEQ ID NO: 478 - DNA, 20 bp, Homo Sapiens
acaaaggaactgatgccctc

SEQ ID NO: 479 - DNA, 20 bp, Homo Sapiens
cctccccacatccatggtac

SEQ ID NO: 480 - DNA, 18 bp, Homo Sapiens
ctgacgagggcacacaga

SEQ ID NO: 481 - DNA, 20 bp, Homo Sapiens
attctcccattgcacagcct

SEQ ID NO: 482 - DNA, 20 bp, Homo Sapiens
ttctgtcatccatgctcccc

SEQ ID NO: 483 - DNA, 20 bp, Homo Sapiens
aagctacagccaggtcactt

SEQ ID NO: 484 - DNA, 20 bp, Homo Sapiens
tacctggaggatgatggctg

SEQ ID NO: 485 - DNA, 20 bp, Homo Sapiens
atctgggaccaagagtagcc

SEQ ID NO: 486 - DNA, 19 bp, Homo Sapiens
ctgaatgaggcagggaagc

SEQ ID NO: 487 - DNA, 20 bp, Homo Sapiens
acatccccgtgtcactactg

SEQ ID NO: 488 - DNA, 20 bp, Homo Sapiens
attccctgcacttctaggca

SEQ ID NO: 489 - DNA, 23 bp, Homo Sapiens
cagagtcacaaaataacacccca

SEQ ID NO: 490 - DNA, 20 bp, Homo Sapiens
gccaggtgaaagcacacgta

SEQ ID NO: 491 - DNA, 18 bp, Homo Sapiens
atctacctgccctgcacg

SEQ ID NO: 492 - DNA, 18 bp, Homo Sapiens
cacaggctgtggaggtcc

SEQ ID NO: 493 - DNA, 20 bp, Homo Sapiens
cactagagtggtgcagccta

SEQ ID NO: 494 - DNA, 19 bp, Homo Sapiens
gtaccagccccaagtggat

SEQ ID NO: 495 - DNA, 20 bp, Homo Sapiens
gtctcccattctctgcctct

SEQ ID NO: 496 - DNA, 20 bp, Homo Sapiens
ctgactggggtccacaaact

SEQ ID NO: 497 - DNA, 20 bp, Homo Sapiens
cattcccagctaccctcctc

SEQ ID NO: 498 - DNA, 24 bp, Homo Sapiens
tcttaaagcaattaaggagcacct

SEQ ID NO: 499 - DNA, 19 bp, Homo Sapiens
cagcattgtcctcaggcac

SEQ ID NO: 500 - DNA, 21 bp, Homo Sapiens
ataagagcatgaccctgcatg

SEQ ID NO: 501 - DNA, 19 bp, Homo Sapiens
caggagagtgtgcactggg

SEQ ID NO: 502 - DNA, 19 bp, Homo Sapiens
acaggtgtccccagagatg

SEQ ID NO: 503 - DNA, 20 bp, Homo Sapiens
ctgaggcagggcatgatact

SEQ ID NO: 504 - DNA, 19 bp, Homo Sapiens
cacctcacctgagtcccag

SEQ ID NO: 505 - DNA, 18 bp, Homo Sapiens
ccgccacgagctcagaag

SEQ ID NO: 506 - DNA, 20 bp, Homo Sapiens
tctccccatgacagccattt

SEQ ID NO: 507 - DNA, 20 bp, Homo Sapiens
ctcctcaggcatgggttctt

SEQ ID NO: 508 - DNA, 18 bp, Homo Sapiens
gtggcaagtggctcctga

SEQ ID NO: 509 - DNA, 20 bp, Homo Sapiens
ccctaccctgcctcaacata

SEQ ID NO: 510 - DNA, 24 bp, Homo Sapiens
aagtatacccaaccattcaactct

SEQ ID NO: 511 - DNA, 20 bp, Homo Sapiens
tacattctcccaaccccacc

SEQ ID NO: 512 - DNA, 20 bp, Homo Sapiens
tggtgatgtgcagtcaacag

SEQ ID NO: 513 - DNA, 18 bp, Homo Sapiens
ggcctgtctgtgtgctca

SEQ ID NO: 514 - DNA, 19 bp, Homo Sapiens
gagccacccacttcaggag

SEQ ID NO: 515 - DNA, 20 bp, Homo Sapiens
agggtgggtggaagtttagt

SEQ ID NO: 516 - DNA, 19 bp, Homo Sapiens
gagacacggttgggagagg

SEQ ID NO: 517 - DNA, 20 bp, Homo Sapiens
cccacctacacattccctca

SEQ ID NO: 518 - DNA, 20 bp, Homo Sapiens
cagcttcctatgcccagagg

SEQ ID NO: 519 - DNA, 18 bp, Homo Sapiens
ctgagcgtggtggcagtc

SEQ ID NO: 520 - DNA, 18 bp, Homo Sapiens
ctgtccctgctcgtcaca

SEQ ID NO: 521 - DNA, 20 bp, Homo Sapiens
cgtacccagaagacaatggc

SEQ ID NO: 522 - DNA, 24 bp, Homo Sapiens
ggctttgaaatggaactgaaaact

SEQ ID NO: 523 - DNA, 20 bp, Homo Sapiens
ccaagagtccccacatctgg

SEQ ID NO: 524 - DNA, 20 bp, Homo Sapiens
atggggttctccttgggaag

SEQ ID NO: 525 - DNA, 20 bp, Homo Sapiens
ggggtagccaggaagatctc

SEQ ID NO: 526 - DNA, 20 bp, Homo Sapiens
ctgcagcacttctttgtcca

SEQ ID NO: 527 - DNA, 19 bp, Homo Sapiens
gtgagggagggaaaggcag

SEQ ID NO: 528 - DNA, 20 bp, Homo Sapiens
tacacctcccctcttggaac

SEQ ID NO: 529 - DNA, 20 bp, Homo Sapiens
ctgaggggcaatagggaagg

SEQ ID NO: 530 - DNA, 20 bp, Homo Sapiens
gcactcggcagatctcagta

SEQ ID NO: 531 - DNA, 20 bp, Homo Sapiens
tcatcccttccatcacctcc

SEQ ID NO: 532 - DNA, 20 bp, Homo Sapiens
gagccctgttcttgctgatc

SEQ ID NO: 533 - DNA, 20 bp, Homo Sapiens
gcgccctatgaccttcacta

SEQ ID NO: 534 - DNA, 21 bp, Homo Sapiens
cagagtgtgcctaggaagttg

SEQ ID NO: 535 - DNA, 20 bp, Homo Sapiens
attcgcccgtagattgaccc

SEQ ID NO: 536 - DNA, 18 bp, Homo Sapiens
ccacagggacaagggctg

SEQ ID NO: 537 - DNA, 20 bp, Homo Sapiens
tgggattcgaaccaccaaac

SEQ ID NO: 538 - DNA, 19 bp, Homo Sapiens
gacaccaacccgtctaccc

SEQ ID NO: 539 - DNA, 20 bp, Homo Sapiens
ccaccttgcatgggtactca

SEQ ID NO: 540 - DNA, 20 bp, Homo Sapiens
acaaccttaggttccaagcc

SEQ ID NO: 541 - DNA, 19 bp, Homo Sapiens
gaggccccaggaagaatcc

SEQ ID NO: 542 - DNA, 19 bp, Homo Sapiens
ccctgcctctgtgtgtctg

SEQ ID NO: 543 - DNA, 19 bp, Homo Sapiens
ccatgcctggaactgcttc

SEQ ID NO: 544 - DNA, 18 bp, Homo Sapiens
catctccaccacccaggg

SEQ ID NO: 545 - DNA, 19 bp, Homo Sapiens
ctgaggctggccacttgaa

SEQ ID NO: 546 - DNA, 19 bp, Homo Sapiens
ccaaaggccaaaggaggtc

SEQ ID NO: 547 - DNA, 18 bp, Homo Sapiens
aaggctgcctgggacatc

SEQ ID NO: 548 - DNA, 19 bp, Homo Sapiens
tccccttccctgactccag

SEQ ID NO: 549 - DNA, 18 bp, Homo Sapiens
gacacaggctggagctcc

SEQ ID NO: 550 - DNA, 18 bp, Homo Sapiens
ccagggggagaaggacct

SEQ ID NO: 551 - DNA, 20 bp, Homo Sapiens
ccaagccgcttaatccttcc

SEQ ID NO: 552 - DNA, 20 bp, Homo Sapiens
tgcccccagaatgacaacta

SEQ ID NO: 553 - DNA, 20 bp, Homo Sapiens
aatctcagaccccacccttc

SEQ ID NO: 554 - DNA, 20 bp, Homo Sapiens
cccaccttgaacacgcaaat

SEQ ID NO: 555 - DNA, 20 bp, Homo Sapiens
cctcctctactgctaaggcc

SEQ ID NO: 556 - DNA, 20 bp, Homo Sapiens
gaccgcaaagccggtactta

SEQ ID NO: 557 - DNA, 20 bp, Homo Sapiens
cacccttttcccgtctgaag

SEQ ID NO: 558 - DNA, 19 bp, Homo Sapiens
gacctcagaccgaagtccc

SEQ ID NO: 559 - DNA, 18 bp, Homo Sapiens
agggaagggtgcaggtag

SEQ ID NO: 560 - DNA, 19 bp, Homo Sapiens
atatgtggggagcatgcgt

SEQ ID NO: 561 - DNA, 19 bp, Homo Sapiens
gctccaggcctttgtctta

SEQ ID NO: 562 - DNA, 20 bp, Homo Sapiens
tcaaaggcggccaaagaatt

SEQ ID NO: 563 - DNA, 20 bp, Homo Sapiens
cccactttctccccctcaat

SEQ ID NO: 564 - DNA, 19 bp, Homo Sapiens
ttctacacgaccaggccag

SEQ ID NO: 565 - DNA, 18 bp, Homo Sapiens
cctgaaccctggaccctg

SEQ ID NO: 566 - DNA, 18 bp, Homo Sapiens
cgaagtcctgggagcccc

SEQ ID NO: 567 - DNA, 20 bp, Homo Sapiens
tcggatggctacagtctgtg

SEQ ID NO: 568 - DNA, 20 bp, Homo Sapiens
cagacctgggtggctatgag

SEQ ID NO: 569 - DNA, 18 bp, Homo Sapiens
cagcaagcctggccatgg

SEQ ID NO: 570 - DNA, 18 bp, Homo Sapiens
tcctccccaactcccact

SEQ ID NO: 571 - DNA, 20 bp, Homo Sapiens
ccagagagtagaacagggca

SEQ ID NO: 572 - DNA, 19 bp, Homo Sapiens
ctggcctcacactgtctgg

SEQ ID NO: 573 - DNA, 20 bp, Homo Sapiens
gtaaaaactgcacccagcct

SEQ ID NO: 574 - DNA, 18 bp, Homo Sapiens
tcacccctaggcccatga

SEQ ID NO: 575 - DNA, 18 bp, Homo Sapiens
agtctccggagccccatg

SEQ ID NO: 576 - DNA, 19 bp, Homo Sapiens
cctctatatccccgccccc

SEQ ID NO: 577 - DNA, 18 bp, Homo Sapiens
cacctgtgcccgctccta

SEQ ID NO: 578 - DNA, 18 bp, Homo Sapiens
agggttccgtggggactc

SEQ ID NO: 579 - DNA, 18 bp, Homo Sapiens
taccaggcagggttggtg

SEQ ID NO: 580 - DNA, 18 bp, Homo Sapiens
cgtcgttgtctccccgaa

SEQ ID NO: 581 - DNA, 19 bp, Homo Sapiens
ctgcttccccaccatcctg

SEQ ID NO: 582 - DNA, 20 bp, Homo Sapiens
gtatgggctcagctgcaatt

SEQ ID NO: 583 - DNA, 20 bp, Homo Sapiens
ttgtggggtaggacagtgac

SEQ ID NO: 584 - DNA, 20 bp, Homo Sapiens
ctcgacaaagcaacaggtcc

SEQ ID NO: 585 - DNA, 20 bp, Homo Sapiens
agtgcaaggtcacagaggtc

SEQ ID NO: 586 - DNA, 20 bp, Homo Sapiens
aaatgagcctctcagtgccc

SEQ ID NO: 587 - DNA, 19 bp, Homo Sapiens
ctctctgggggctgagact

SEQ ID NO: 588 - DNA, 18 bp, Homo Sapiens
cacccacgaaaacccacc

SEQ ID NO: 589 - DNA, 19 bp, Homo Sapiens
tctgcgaagtcctgggaag

SEQ ID NO: 590 - DNA, 20 bp, Homo Sapiens
taacttccatcagaggcgct

SEQ ID NO: 591 - DNA, 20 bp, Homo Sapiens
atgcatctaaagccccgaga

SEQ ID NO: 592 - DNA, 19 bp, Homo Sapiens
catcctcccccagtgtctg

SEQ ID NO: 593 - DNA, 18 bp, Homo Sapiens
cacacacagggcccactg

SEQ ID NO: 594 - DNA, 20 bp, Homo Sapiens
gacttttcgagggcctttcc

SEQ ID NO: 595 - DNA, 19 bp, Homo Sapiens
gggcagacggggaaactta

SEQ ID NO: 596 - DNA, 19 bp, Homo Sapiens
ctgtcacaggccaagggag

SEQ ID NO: 597 - DNA, 20 bp, Homo Sapiens
caggtctttaggaggagggg

SEQ ID NO: 598 - DNA, 19 bp, Homo Sapiens
ctctagctggccggtcttc

SEQ ID NO: 599 - DNA, 20 bp, Homo Sapiens
tttccaacccctccctactc

SEQ ID NO: 600 - DNA, 20 bp, Homo Sapiens
ttttacgcgtggaatgcaca

SEQ ID NO: 601 - DNA, 20 bp, Homo Sapiens
aagagggaaaagttgccact

SEQ ID NO: 602 - DNA, 18 bp, Homo Sapiens
ccctcgcctccctcactg

SEQ ID NO: 603 - DNA, 20 bp, Homo Sapiens
gcgtatgatggaggcgtagt

SEQ ID NO: 604 - DNA, 18 bp, Homo Sapiens
aggatggccgcagagatg

SEQ ID NO: 605 - DNA, 19 bp, Homo Sapiens
cagacctctcctccagcct

SEQ ID NO: 606 - DNA, 19 bp, Homo Sapiens
caaagcctcgcacacactc

SEQ ID NO: 607 - DNA, 20 bp, Homo Sapiens
gtaacgattgcccagtgctc

SEQ ID NO: 608 - DNA, 19 bp, Homo Sapiens
caccccagcgcactagtta

SEQ ID NO: 609 - DNA, 143 bp, Homo Sapiens
gctcatttttgttaatggtggctttttgtttgtttgttttgttttaaggtttttggattcaaagcataaaaaccattacaagatatacaatctgtaagtatgttttcttatttgtatgcttgcaaatatcttctaaaacaact

SEQ ID NO: 610 - DNA, 143 bp, Homo Sapiens
gaacaatgaataaaccattttgtctcattaaaattttagattattatgtagttggcagctgagaacaatacttagtggataccatcgaatagtacaacaggtaagtcctttttaaaaggtttatgttttcagtgaagataaga

SEQ ID NO: 611 - DNA, 160 bp, Homo Sapiens
atcatgctgacgcttctcctttatcttttaaaatttgcagtggctgagaggactactaactagtagacagagttttaacatcatatttggtgaatgtccatattgtagtaaggtaagcaaattgttaatcacatctcataaaatgtgcctagctttcagt

SEQ ID NO: 612 - DNA, 241 bp, Homo Sapiens
tgcagatttttaaaaagtctcttttccattattttttcaacttataggaatgaggcaaagtagcctaaagaaagattggttcttatcagaagaagaatttaaattatggaacagactttatagattaagggacagtgatgaaattaaagagataacattgcctcaagttcagttttcttctttacaaaatgaggaaaacaaaccagtaagttgaatatattttcagatgttcttttccccc

SEQ ID NO: 613 - DNA, 104 bp, Homo Sapiens
agttaataaggacatggtttctgttctttttttacagatacttttaaagttttgtcagaaaagagccactttcaaggtaggacaagtttggaaatgtattctca

SEQ ID NO: 614 - DNA, 173 bp, Homo Sapiens
aggaaactagagttcattttccttttcttaggacctgttatggaatttgattatgtaatatgcgaagaatgtgggaaagaatttatggattcttatcttatgaaccactttgatttgccaacttgtgataactgcaggtacttattttagatggtgttcttaattgctaatgt

SEQ ID NO: 615 - DNA, 209 bp, Homo Sapiens
tcgcaagtctgaatcacaacttatttaaatatggattttgtgttgtagattgtgaagaggtctcttgaagtttggggtagtcaagaagcattagaagaagcaaaggaagtccgacaggaaaaccgagaaaaaatgaaacagaagaaatttgataaaaaagtaaaaggtagatggccacattttatatcgtgaaggattgtgttttacca

SEQ ID NO: 616 - DNA, 192 bp, Homo Sapiens
tgtgcattgagagtttttatactagtgattttaaactataatttttgcagaatgtgaaaagctatttttccaatcatgatgaaagtctgaagaaaaatgatagatttatcgcttctgtgacagacagtgaaaacacaaatcaaagagaagctgcaagtcatggtaagtcctctgtttagttgaactacaggt

SEQ ID NO: 617 - DNA, 332 bp, Homo Sapiens
ccaggttagctggtaagaggatttttttggagaaaaaaatgatatttagaaagttaatttctaattccggaatggaataaaaacaatatgagtagtgtaatcttgtagaaaaagagttgtataatcttgtagaatttctcattctgtggtacaacccaggggtaaactattattccagtagtcagtacacttttctagataaatcttgagtgaaaaccagcaatttctttttccttgtggtctgattcctttttctaatccatgaaggccatcttgtagattacatttatcattaatgcaagaataaagacaattcctcctgtcagttgcgt

SEQ ID NO: 618 - DNA, 155 bp, Homo Sapiens
aagcttttcaggataatttctgtttttttttgtttgtttgtttttaggagttatggtacagcacctgtaaatcttaacatcaagacagggggaagagtttatggaactacaggtaaaatttgtattttctgttgcatcaatagggaaataaggca

SEQ ID NO: 619 - DNA, 212 bp, Homo Sapiens
aggatgatactggttgacacaattgttttattttatttcagttggttagaagcaaacgctgaatatcttgtagaaagagattatgaatcagcttgtaaaatatggagtggaaatgaaatgctcttaactttacacaaaatgggtatcaccactgctacttttcccattttgcaggtaagatattttttctacctgtgaaacgtatttagtga

SEQ ID NO: 620 - DNA, 151 bp, Homo Sapiens
tcagcttttccttaaagtcacttcatttttattttcagtgaagaactgttctaccagatactcatttatgattttgccaattttggtgttctcaggttatcggtaagtttagatccttttcacttctgaaatttcaactgatcgtttctga

SEQ ID NO: 621 - DNA, 150 bp, Homo Sapiens
caccatatattaacttctgacatttgcaaatttcaggagttgtcacagcagaaatgtttagacatatgcagaactctgagataattcgaaaaatgactgaagaattcgatgaggtaacttactaccttaagtgttttgataacttatgca

SEQ ID NO: 622 - DNA, 150 bp, Homo Sapiens
gctacaaaagagctcaacaatttttttattacgtgcaatttttttaataggaataaaaaaatacgttgttggcctcattatcaagacgtcatctgacccaacttgtgtagaggtaagagtttattttggagcttattgggagagcataaa

SEQ ID NO: 623 - DNA, 146 bp, Homo Sapiens
gtgattttctaaaatagcaggctcttatttttctttttgtttgtttgtagcgatacaaacttggagttcgcttgtattaccgagtaatggaatccatgcttaaatcagtaagttaaaaacaatataaaaaaatttcagccgggcgc

SEQ ID NO: 624 - DNA, 128 bp, Homo Sapiens
tcaccactgagcaaatgtttgaaattatgttaattttgacaggtacaaaatcaacatgcaaaagaagagtctcttgctgatgatctttttaggtaaagtttgattcacctttctcatgtacctttgag

SEQ ID NO: 625 - DNA, 199 bp, Homo Sapiens
agcagttgtgattctttctttctacttgtgtgatttacaggattaaagacaacaactccaggaccaagcctttcacaaggcgtgtcagttgatgaaaaactaatgccaagcgccccagtgaacactacaacatacgtagctgacacagaatcagagcaagcagatacatggtaaagcttcttcattaccgtactattgt

SEQ ID NO: 626 - DNA, 160 bp, Homo Sapiens
ttggaagtataatagcagttcttttctctttataggttagaccaaagccattgcttttgaagttattaaagtctgttggtgcacaaaaagacacttatactatgaaagaggtaagctgaatcaagagataagtagtatctcactagttacatgtagccat

SEQ ID NO: 627 - DNA, 177 bp, Homo Sapiens
tgacagctatgctaatagtgtttcttgtctatataattgcagatctctacaatatggaaatcagttcatatatcagtcaatgccacgaatgttaactctatggcttgattatggtacaaaggcatatgaatgggaaaaaggtataactcttcacgtaaaagttttaaaggactagga

SEQ ID NO: 628 - DNA, 159 bp, Homo Sapiens
tgggtgcttgggtgtgtataaacacatgatactgtatcatagcaataagatttgtaaaacattgcaatggctgaaaaactgtctaacaggaaattttaagtgttattccaaagaagaacaagcctaaaagtaagttaacctttcagagtggttgaaagt

SEQ ID NO: 629 - DNA, 176 bp, Homo Sapiens
tctgtcttctcctctcttcctttacacaaacttaaacagaatggaaatgaaaaccaaggagaagttgaagaacaaacatttaaagaaaaggaattagacagaaaacctgaagatgtgcctcctgagattttgtctaatgaaaggtatacaaaatgtgtactttttcagtgcaaagt

SEQ ID NO: 630 - DNA, 150 bp, Homo Sapiens
tggttaggagaatgagttgttgttgttgatgttgttttttaaccacacagacctttccaaataaaagattccagttgcatatgaaatattagatcacaagtacagtaagtaatatttctctaacatgtcatccctcttgaaggagctgtc

SEQ ID NO: 631 - DNA, 152 bp, Homo Sapiens
tgcatctgtggcattaaatggtgatacatattatttgaatttcagatttacggcaagatatgctaacacttcaaattattcgtattatggaaaatatctggcaaaatcaaggtcttgatcttcggtaggtaaccagtaaggcaacctgtatg

SEQ ID NO: 632 - DNA, 108 bp, Homo Sapiens
atggtttttatgacacagagttgtgattttttttctttttcacagtttctcaagcaagacctcccccaaatcagaagaaaggtgaggttgtgcatatgattttaaact

SEQ ID NO: 633 - DNA, 161 bp, Homo Sapiens
aggatcactttatatggatcactttttcttattttgtagtcttcaaaaattaaaaaaggaagcaaaggggatacatccatgttgaaaccaacactgatggcagcagttccggtaagaagtgacccttatttaatattgagtattaaagaagtatcacccgc

SEQ ID NO: 634 - DNA, 158 bp, Homo Sapiens
tgtgtacatggtgccagaatatttgtttttcttcttatagaatgtccaacatcccagcttgcttccttggatcagcacagtcagaaaatgttctaacagatattaaattgtgagtaatttttttccctcaacttttattttggatttatgggggtgca

SEQ ID NO: 635 - DNA, 200 bp, Homo Sapiens
agtcaatttttctttcttctcttgcaggtgaacctatgggtcgtggaacaaaagttatcctacacctgaaagaagaccaaactgagtacttggaggaacgaagaataaaggagattgtgaagaaacattctcagtttattggatatcccattactctttttgtaagtttttatgtaattgcagagtgaatttctgtctgt

SEQ ID NO: 636 - DNA, 150 bp, Homo Sapiens
ttggaggccactgctatggcttatgaaaataattgttttttgttttacagtgggcaaatcaaactagcagattttggacttgctcggctctataactctgaagagaggtaaggcattaattaaaattacatgtgggaaataaggtttgtt

SEQ ID NO: 637 - DNA, 194 bp, Homo Sapiens
aaatgtattcactgtcttctctttctttaggttccagcaacaaattatatatatacacccctgaatcaacttaagggtggtacaattgtcaatgtctatggtgttgtgaagttctttaagcccccatatctaagcaaaggaactggtaggtattaaaactggtggagttttttggagtggaaatgcattattga

SEQ ID NO: 638 - DNA, 154 bp, Homo Sapiens
tgtgtgactctaaattgactgcattaattttctcactctcgtcttgcagcattttcagttagctttggttgactgtaatccctgcactttgtccaatgctgaaagtaagtattattaagtactgtagttttctacatgtattccgatcacttca

SEQ ID NO: 639 - DNA, 211 bp, Homo Sapiens
tgtgtgacatgttctaatatagtcacattttcattatttttattataaggcctgctgaaaatgactgaatataaacttgtggtagttggagctggtggcgtaggcaagagtgccttgacgatacagctaattcagaatcattttgtggacgaatatgatccaacaatagaggtaaatcttgttttaatatgcatattactggtgcaggacc

SEQ ID NO: 640 - DNA, 183 bp, Homo Sapiens
atgcaaagtacctaactccactgatttctttttccctcactttttaggattatggctgctgttcctcaaaataatctacaggagcaactagaacgtcactcagccagaacacttaataataaattaagtctttcaaaaccaaaattttcgtaagtgttttgactggtttgctgtcacataggc

SEQ ID NO: 641 - DNA, 161 bp, Homo Sapiens
tgtttgtgcctcactttgcaggagttccactatatagaagaagatctttatcgaacaaagaacacattgcaaagcagaattaaagatcgagacgaagaaattcaaaaactcaggaatcaggtatgaatcactattcacaacttgtgaaaagatgccactga

SEQ ID NO: 642 - DNA, 150 bp, Homo Sapiens
acacgtcttggggatatcacttttgttatttttatttttagggaagcacactgagaaagcggaagatgtatgaggaattccttagtaaagtctctattttaggtgagttgtaaagtgtgttaactttgctagtatgtgagatacccctga

SEQ ID NO: 643 - DNA, 155 bp, Homo Sapiens
actggtatggaaatattacagtcctgtaattctttcttctaggtcatattgaacattccagatacctatcattactcgatgctgttgataacagcaagatggctttgaactcagtaagtggttaattattaccttcctggccttttctttgttcc

SEQ ID NO: 644 - DNA, 198 bp, Homo Sapiens
gccatgttttacatttgagttcacagaaaggaaatgtttattctaggtctgcttcgcctgtgtagatgggaaagaattccgtcttgctcagatgtgtggacttcatattgttgtacatgcagatgaattagaagaacttatcaactactatcaggtattaacgagacttttatatgacctgagatcttttaccataga

SEQ ID NO: 645 - DNA, 160 bp, Homo Sapiens
acaaggctgagacctgagttgataaaatttctttgttctttcagtgaagagaaaggaagtacagaaaacatgcagaaagcacagaaaggaaaaccaaggttctcatgaatctccaactttaaatcctgtaggtattgaaataggtatcagctttccttga

SEQ ID NO: 646 - DNA, 173 bp, Homo Sapiens
tgtcactttgttctgtttgcaggtggaaaaccatgaattccttgtaaaaccttcatttgatcctaatctcagtgaattaagagaaataatgaatgacttggaaaagaagatgcagtcaacattaataagtgcagccagagatcttggtaagaatgggtcattggaggttggaa

SEQ ID NO: 647 - DNA, 135 bp, Homo Sapiens
tggctgttgtcactattgcatatgctaactttttctgtttacatttcagggcatttgaatatgaaattcgattttacactggaaatgaccctctggatgtttgggataggtgggtctttttatttcacaaggaca

SEQ ID NO: 648 - DNA, 150 bp, Homo Sapiens
gctgtttctcttttctccaccattctataggaataagatggtagaatacctgacagactgggttatgggaacatcaaaccaagcagcagatgatgatgtaaaatgtcttacaaggtaaaaaaagaatgaccttcaagtattagtgggttt

SEQ ID NO: 649 - DNA, 150 bp, Homo Sapiens
actgtgtattcatgttcccctttctagtgctgattataaacctaagaaaattaaaacagaagataccaagaaggagaagaaaagaaaactagaagaagaagaggttagtaaagagacttaggtcctttggggcttgagtttggaagtggg

SEQ ID NO: 650 - DNA, 150 bp, Homo Sapiens
ggatttaactttgtttttctctgcctgattgggttctctctttattttagtttctacagagcctgtggagacctctcgatggacagaagaagaaatggaagttgctaaaaaaggtaaattgtagtagttctggtttctcaggtttttgtt

SEQ ID NO: 651 - DNA, 158 bp, Homo Sapiens
agacttcgagtgtttaaatgaaagattaaagtctcaatacttttttaggtacaatggtggctgttgcaattagcccaggaactagaggagagactgactaaagaccgaaatgatgtaagattttctttctttattcctggggtgggctttgcaattta

SEQ ID NO: 652 - DNA, 128 bp, Homo Sapiens
tcagaagttctggaaatacttcatttatttttaaatccttttgttttaggctctccagcagaactatctcctactactctttcccctgttaatcatagcttgggtaagttgcacatatgttcccctca

SEQ ID NO: 653 - DNA, 152 bp, Homo Sapiens
atgcttcagatgttgtatgtaatgtattctttttattttatgtgtagatggctcttggacaagtccgagcagtacaacacactgggagggaatgccctctccttttaaaggcaggaatttttatttattacctgtgttcagtatgtaaacgt

SEQ ID NO: 654 - DNA, 133 bp, Homo Sapiens
ctactcatgcccctcaaacttatttttaataatttcttttcccttcacagctatttgcatgcaaagaacatcatccatagagacatgaaatccaacagtatcctttggttgttgagttcatttgactgctcgg

SEQ ID NO: 655 - DNA, 151 bp, Homo Sapiens
tcttaaatgatcctcttctcccagataatagatgccactcaaaaaggaaattgctctcgtttcatgaatcacagctgtgaaccaaattgtgaaacccaaaaagtaagttgaggtggatttagagtttgaggtatttgttcacgattgctgt

SEQ ID NO: 656 - DNA, 151 bp, Homo Sapiens
gcgatgtgcatatataatggaaaggtttttgttattttcagggtccaccaatgagctgtgtacgattggctgaaagagttgtagctctcatttgctgtgagaaactgcacaaaattggtaaggatgtttgaaaagcatatacgaatgaaaa

SEQ ID NO: 657 - DNA, 151 bp, Homo Sapiens
aatcctgtttgcagcgtgagttaacctgcaactgattttgttttacagatggttttatcattagcgtctgaactcagagagaatcatcttaatggatttaacactcaaaggcggtaggtgttaaactaaacatccttcttctcaggtttca

SEQ ID NO: 658 - DNA, 151 bp, Homo Sapiens
actccattcagaaagtaattttcacctttttttttttttcaaggaaactgagaagaaaatatggcacttcaaatatcctatcttcttcctgtgtatagggctagacttacaggtagagtgaagctatgggaccaggtcacagtgaagtcct

SEQ ID NO: 659 - DNA, 171 bp, Homo Sapiens
tcaggatttttcctttctctctcctattattagacttattcgtctaatggaagagatcatgagtgagaaggagaataaaaccattgtttttgtggaaaccaaaagaagatgtgatgagcttaccagaaaaatgaggagagatgggtatgtgtgagctcctccattgaagca

SEQ ID NO: 660 - DNA, 339 bp, Homo Sapiens
gagttctaggctactgtggctttttccagtagatttagatgagattatgtgttttgaaatgttttgtgggatcccttagaaagcatcacttcagggcagagacactcaatattgccagccagcttgggttctaaagtgatttaatcaaattcatgctcctgatcttttttttcccccttcctttggctatgaaaacccaaagcccggagtgattgttttctccttgctttaagcagtgaagttatcctaatgcaaaagagcttagtagaaaatgagtggtttacctttttttctaaaagtatattttcaagtttattctggaatgtgatgtcttggtcc

SEQ ID NO: 661 - DNA, 176 bp, Homo Sapiens
gtgaatacactttctgctggttttaaatgacagatactgaaataaaaataaacatcaaacaagaaagtgcagatgtaaatgtgattggaaacaaggatgtcgttactgaagaggatttggatgtttttaagcaggcccaggaactttcttgggaggtaaggcgaggatcccacatt

SEQ ID NO: 662 - DNA, 159 bp, Homo Sapiens
aaccaagtcagtaaggccatatacagttattatgttttttactctcaggggaaagttggggacatgctgctacaatacggctaatctttcattgggaccgaaagcaaaggtcagtacagaaacaagttaataactccgaatattgggttaattatactg

SEQ ID NO: 663 - DNA, 151 bp, Homo Sapiens
aaacccttctgtttctttcacagatgagtgccaaaccaaatatggaaatgctaatgcctggagatactgtaccaaagtttttgacatgctcacagtagcagctgtaagtttctatttttaaagtctcatgtacgttcctgccaataacaca

SEQ ID NO: 664 - DNA, 164 bp, Homo Sapiens
tcctgtgagtgttctgtatgttaacacttttattccttgttttgttttaggcgataaactacattcagttgagtctgcaagactgggaggaactggggtgataagaaatctattcactgtcaaggtgagaattagcaaattttcccccttcttctgtactttct

SEQ ID NO: 665 - DNA, 161 bp, Homo Sapiens
gctgggaacatttgtcatttattcttttctactccttgtattttgtgcaggtctgcagactcgtgaatgaggtctaccacatgtataatcgacaccagtatccatttgttgttcttaacatttctgttgattcaggtaagttccattggcatttcagtaca

SEQ ID NO: 666 - DNA, 124 bp, Homo Sapiens
tgccgtttcgagaattttattcacttttatatttatgtctcacatctagggaactagctcttcagaaaaatccaagtcttcaggatcgtcacgatcaaagaggttggttgatgttgaagggaca

SEQ ID NO: 667 - DNA, 155 bp, Homo Sapiens
tgcacactgaaattaggacgtttatatttcttcaggtattagaaaactactcggatgctccaatgacaccaaaacagattctgcaggtcatagaggcagaaggactaaaggaaatgaggtttgtattgttcttgttgcttaacatgagggtttca

SEQ ID NO: 668 - DNA, 150 bp, Homo Sapiens
tttttcccccttgatccttctaggtggggacggatggcctgttgcgtctcagcagcagtgcactaaataacgagttttttacccatgcggctcagagctggcgggagcgcctggctgatggtatgtagacttggtcatctcggacggctt

SEQ ID NO: 669 - DNA, 152 bp, Homo Sapiens
acttattgagcatgcctggttttttgtcttccagcaatatccagattattatgcaataattaaggagcctatagatctcaagaccattgcccagaggatacaggtatgaagatgaccataagtaaatgattgtggtttagagcagattggcc

SEQ ID NO: 670 - DNA, 162 bp, Homo Sapiens
acgcagtgctaaccaagttctttcttttgcacagggcattttggttgtgtatatcatgggactttgttggacaatgatggcaagaaaattcactgtgctgtgaaatccttgaacagtaagtggcattttatttaaccatggagtatacttttgtggtttgca

SEQ ID NO: 671 - DNA, 100 bp, Homo Sapiens
ttttatatgatctttcctggttggcaggacccatggatgaaggaccagatcttgatctaggtaattttgaattctagttgtgcttcatatcgtgctttgt

SEQ ID NO: 672 - DNA, 163 bp, Homo Sapiens
aagaatgcctgggactgaggggagatatttttgtttgtcagagtcagagcactttttccgatgctgtttggataaaaaatcacaaagaacaatgcttgctgttgtggactacatgagaagacaaaagaggtaatgtaatgagtgttgcttcttacgtttagga

SEQ ID NO: 673 - DNA, 150 bp, Homo Sapiens
aaagtgtagactaatgatgtgacttttgttttcacagactgaaacagcagagcttcctgcttctgatagcataaacccaggcaacctacaattggtttcagagttaaaggtcagaagaatattctcttccagtgtctcgtgtcttacata

SEQ ID NO: 674 - DNA, 150 bp, Homo Sapiens
tgtactctttttcctgttgctgttcttttctgcaggagggaaaacccctgatcctaaaatgaatgctaggacttacatggatgtaatgcgagaacaacacttgactaaagaagaagtatgtaaacctgtctcctgttttaatggttgtga

SEQ ID NO: 675 - DNA, 151 bp, Homo Sapiens
aagcaaacttgttctgtttttacccactgattctttttcagccccttctcaaagtcagcatgtcaatgagagactgcttgatacttgtccttcggaaagctatgtttgccaagtatgtagcatctttttctatcataggaagacgttgtct

SEQ ID NO: 676 - DNA, 161 bp, Homo Sapiens
tgtgtgtttctgtgggtttctttaaggtttggacagaagggtaaagctattaggattgaaagagtcatctatactggtaaagaaggcaaaagttctcagggatgtcctattgctaagtgggtaagtgtgacttgataaagcctttggtcttaaatcttggg

SEQ ID NO: 677 - DNA, 150 bp, Homo Sapiens
tgtttttgtccctctctcttgcagtgaaattacagacaacccttacatgacgtcaatccctgtgaatgcttttcagggactatgcaatgaaaccttgacactgtgagtattaccagttctactccctccatcaactaaattctattttga

SEQ ID NO: 678 - DNA, 169 bp, Homo Sapiens
acatactttgtatcatcttattggcagcactggaagaagctgcaaaacgtttccaggaattgaaagcacaaagagaaagtaaagaagccctagagattgaaaaaaactcaagaaaaccccctccctacaaacacatcaaagtaagtctttatctctggcctgggattgc

SEQ ID NO: 679 - DNA, 159 bp, Homo Sapiens
tgttttcctttgtgtcattcccttttatcaggttgcccacattcccaaatcagatgctttgtactttgatgactgcatgcagcttttggcgcagacattcccgtttgtagatgacaatgaggtgaggtataaaataacctggttaatagaaaaactcca

SEQ ID NO: 680 - DNA, 166 bp, Homo Sapiens
ggattcagtgaggaatgctttcatgaagttggtgtatctttttaaataggaaaatccttgtaaatgatggtgacgcttcaaaagccagactggaactgagggaagagaatcccttgaaccacaacgtggtaagagattaatagcttctgttgatgccatatctgca

SEQ ID NO: 681 - DNA, 163 bp, Homo Sapiens
acacagaatttgttaagcaacgtagtctttcttttaaattctctttcaggtttttcatatgaaaaagatccccgattatactttgacgacacttgtgttgtgcctgagagactggaaggtaagtagccccatccaaggtttgttgccaggtagaggtttggag

SEQ ID NO: 682 - DNA, 133 bp, Homo Sapiens
tctcatcataccactattattttgcagttttgtgtgcgacaactgcttgaagaaaactggcagacctcgaaaagaaaacaaattcagtgctaagagtaagtttcgggaagctttctgtttcctggactgcaca

SEQ ID NO: 683 - DNA, 182 bp, Homo Sapiens
acacagccttctcaacctctttttctttttttctttcttgtttttagtctttttgctaaagaacatctgcagcacatgacagaaaagcagctgaacctctatgaccgcctgattaacgagcctagtaatgactgggatatttactactgggccacaggtactgggtatgataagcagcataa

SEQ ID NO: 684 - DNA, 150 bp, Homo Sapiens
ctctcggtgtatttctctacttacctgtaataatgcttttgtcttaatagggtggttctcttcccaaagtggaagccaaattcatcaattatgtgaagaattgcttccggatgactgaccaagaggtaactggattttctggggacatga

SEQ ID NO: 685 - DNA, 150 bp, Homo Sapiens
tcactgtgatagccttatctgcttgtttctctttgactttgtagctcgttctccggtttttagtgccatgtttgaacatgaaatggaggagagcaaaaaggtatgtaacaagatgaagacatgtctgtttagccaggtatctagagtcag

SEQ ID NO: 686 - DNA, 150 bp, Homo Sapiens
gttaatcttaacctgtgctttgcctcctgttctgtcttgactttgccagaaaaatcgagttgagcagcaacttcacgagcatttgcaagatgcaatgtccttcttaaaggatgtctgtgaggtactatttcttttagatggtgccttttt

SEQ ID NO: 687 - DNA, 120 bp, Homo Sapiens
actccaacactgttgctcctaattactgttttatcctacttttaggactctggagatgccacatggaaagaaacattctggttggcaagtatcttcttacatgctcttacttgctccaag

SEQ ID NO: 688 - DNA, 122 bp, Homo Sapiens
gccagagtcctttagccctactcaggttaaaatgatgttttgtttttcagttacttacacgccaagtcaatcatccacagagacctcaagagtaatagtatccttcctgaaatttgtctgcg

SEQ ID NO: 689 - DNA, 229 bp, Homo Sapiens
tcctgggtttcttttcaacttgtaatagtgttgtattcttgtctttaggcaagccaaaattccttccggatagaatatgatacctttggtgaactaaaggtgccaaatgataagtattatggcgcccagaccgtgagatctacgatgaactttaagattggaggtgtgacagaacgcatgccagtaagtggcatttgtggaaatgttggctattttggatgaagtaggc

SEQ ID NO: 690 - DNA, 182 bp, Homo Sapiens
tcctgaagtgagatcttacatcctttcttctcataggtgaagagaaggcagagaaaggacttagcgtccagtgactccaggaaaacgacagagaagcttctgaaaacatttttgaaaagacaagccatcaaaactgccttcagaagcaaaaggcaagaggaaaattatagtcgtgttagaga

SEQ ID NO: 691 - DNA, 150 bp, Homo Sapiens
gaccagaaaggctcagttccctgttttctcttcctaacattttagcaagaacagtgatgaaatcaacatacctcgactcattgtcagtcaactaaaatggcttgacagagttgtggatggcaaggtaggcttatggactttatctcttga

SEQ ID NO: 692 - DNA, 150 bp, Homo Sapiens
aaacattgatttggcttttcccatttattattctgtaggttgctatgacccgagagaagtttccagagaagattccatttagactaacaagaatgttgaccaatgctatggaggtgagtggatatcgggaacgagctgcttccaaatggg

SEQ ID NO: 693 - DNA, 176 bp, Homo Sapiens
tgtctccatttcccaccacagggtcatgctctatcagatttcagaagaagtgagcagatcagaattgaggtcttttaagtttcttttgcaagaggaaatctccaaatgcaaactggatgatgacatggtaagacctggtatcttactgagatttagtcctgagacttggttagcca

SEQ ID NO: 694 - DNA, 156 bp, Homo Sapiens
atttactctggattttgctttttcagatactggctttggcactactagtggaggggcatttggaacatctgcatttggttctagcaacaatactggaggcctctttggaaattcacagactaaaccaggtaggggctttatttgtgatataactgg

SEQ ID NO: 695 - DNA, 151 bp, Homo Sapiens
tgagatgtttttgccttcacaggtgattgaagtgggaaaaaatgatgacctggaggactctaagtccttaagtgatgataccgatgtagaggttacctctgaggtatgaatctttagcaagaactattttgcaccagccccatcttcagat

SEQ ID NO: 696 - DNA, 165 bp, Homo Sapiens
tcccccttgtcttaaaccacaggatttattggatcattcgtgtacatcaggaagtggctctggtcttccttttctggtacaaagaacagtggctcgccagattacactgttggagtgtgtcggtaattcttttttttcctttctttgtgggtaatatgcaatgtt

SEQ ID NO: 697 - DNA, 153 bp, Homo Sapiens
ttgacgtgccattctcttgcttcctcttcctcaaaaaggataagcactgttcaaaggatgccctacttgcaggattaaaacaagatgaaccaggacaagcaggaagtcagaagtcttctaccaagtaaggaaaatgagtttacttcctgttgt

SEQ ID NO: 698 - DNA, 150 bp, Homo Sapiens
tttgggacgacttattgcccttcaatttcctcatggccaaaggcttattcatagggcttcttgactaaagcccttggagcactgggtttttcttgaagtatatggtgagttaatgacttgaatctgcaattgggtgattgcctgaattct

SEQ ID NO: 699 - DNA, 157 bp, Homo Sapiens
agagtaacttcaatgtctttattccatcttctctttagggtcggattccagttaaatggatggcaattgaatccctttttgatcatatctacaccacgcaaagtgatgtgtaagtgtgggtgttgctctcttggggtggaggttacagaaacaccct

SEQ ID NO: 700 - DNA, 264 bp, Homo Sapiens
gatctccggttgggattcctgcggattgacatttctgtgaagcagaagtctgggaatcgatctggaaatcctcctaatttttactccctctccccgcgactcctgattcattgggaagtttcaaatcagctataactggagagtgctgaagattgatgggatcgttgccttatgcatttgttttggttttacaaaaaggaaacttgacagaggatcatgctgtacttaaaaaatacaagtaagttctctgcacaggaaattggt

SEQ ID NO: 701 - DNA, 159 bp, Homo Sapiens
gcattttctctgttcaacaagcagaacaggataattcagacaacaacaccatctttgtgcaaggcctgggtgagaatgttacaattgagtctgtggctgattacttcaagcagattggtattattaaggtacttgtggagaggagtgggagctttctgt

SEQ ID NO: 702 - DNA, 151 bp, Homo Sapiens
gtttgtgacataagcagaacgctttgatttggtttctttctacagctccattttcagtccggcagcacacattactctgcgtacaaaacgattgaacaccagattgcagttcaggtaggaaacgcaagagattctgaagcttgaattgtct

SEQ ID NO: 703 - DNA, 155 bp, Homo Sapiens
tgacagccagattcgtctttgttttatagagttgttgcctgcaatctctatccctttgtaaagacagtggcttctccaggtgtaactgttgaggaggctgtggagcaaattgacattggtaagtcagaaaaaccattttagaagactgagaggag

SEQ ID NO: 704 - DNA, 190 bp, Homo Sapiens
tggaagtctgtgagttctctgatctttacttcttttttaggcacacctgttgtccttaactgactttccgggtcatcagcacttcttcagaagtgttccttttccctcccagcaaatatggaagactgactatcctgatattcccagacattctttgctgtgatttgtaagcccgatataaacccttcca

SEQ ID NO: 705 - DNA, 150 bp, Homo Sapiens
atgttcttcctttaggtatagtctcaataacatttcttcccctaggtgctgctgatgtagagaaggtggaggaaaagtcagcaatagatctgacccctattgtggtagaagacaaaggtgggtgtttggagaagttgattgtggttcaga

SEQ ID NO: 706 - DNA, 152 bp, Homo Sapiens
cctgaagcagtccaggacttatgtgaccgtggtctctttttcttctagttgatcataccagggttgtcctacacgatggtgatcccaatgagcctgtttcagattacatcaatgcaaatatcatcatggtaagctttgcttttcacagtgtt

SEQ ID NO: 707 - DNA, 154 bp, Homo Sapiens
agcttaagaaaagtgacgtggtcaatttttttcttaaatagatcactttgccagctgtgtggaggatggatttgagggagacaagactggaggcagtagtccaggtgagagatgttgagatgttgcagatttgaactaaggcattggcagtaga

SEQ ID NO: 708 - DNA, 156 bp, Homo Sapiens
tccttgagtgtaaggcaattaataacttacacttgtctttatgttccagcctgaaagaatagacccaagcgcatcacgacaaggatatgatgtccgctctgatgtctggagtttggggatcacattggtatgtttatgctgattcaaccttgccac

SEQ ID NO: 709 - DNA, 151 bp, Homo Sapiens
gtctgtggattgacttcttttccttttatgttgttctggtttttaaaggcagcagcctccttggaaagacgaaaagcatcctgggttcaggctgacatctgcacttaacaggtacatgggttgtttcctggtaggagtagattttaaagca

SEQ ID NO: 710 - DNA, 125 bp, Homo Sapiens
tgagcctcatttattttctttttctccccccctaccctgctagtctggagttgatcaaggaacctgtctccacaaagtgtgaccacatattttgcaagtaagtttgaatgtgttatgtggctcca

SEQ ID NO: 711 - DNA, 150 bp, Homo Sapiens
tcccttatgttcttcttctctccagatctgttacctaaagcaataaaaaatggccagaggatcagtgtccgatgaggaaatgatggagctcagagaagcttttgccaaagttggtgagtagacctggtaccccaaattgcatcattctct

SEQ ID NO: 712 - DNA, 150 bp, Homo Sapiens
gcactttaatactaacaggaacagccttgaaaatgtcttttctttccagtacaccccaaaaagggagatttggtatactctgagatccagactactcagctgggagaagaagaggaaggtacgtctttgggaagagattctggctgcaaa

SEQ ID NO: 713 - DNA, 154 bp, Homo Sapiens
tgtcctcagtctgtactaaactcaaaccaagttctcatgcattactaggttggagaaacgtacggtaaggatataacctcccggggcaaagacaagccgattgccgtatgtaaaactttcagtccacttcagtttcaagctttctctgttctct

SEQ ID NO: 714 - DNA, 131 bp, Homo Sapiens
agcagatttgtatgaaagcccttacattttttctaggtatgaagtagctccgaggtctgatagtgaagaaagtggctcagaagaagaggaagaggtaagagtgcatttcctggctttcaaggctctcagtg

SEQ ID NO: 715 - DNA, 216 bp, Homo Sapiens
accctgttacacgcttgtaattgactcttctaggtgagcccattggcaggggtaccaaagtgatcctccatcttaaagaagatcagacagagtacctagaagagaggcgggtcaaagaagtagtgaagaagcattctcagttcataggctatcccatcaccctttatgtgagtatggacttttaaatcttttacacttaacgtgcaggatgtttcc

SEQ ID NO: 716 - DNA, 156 bp, Homo Sapiens
actgaatttgttttagggcacattgaatactttactttccttttcctcagcatcaacaacagcaacttgtgattggcggtgaccggatattcagttgcacatccccacatcaatgcactgccaatggtaagactctccaactcccaatgtcagtgt

SEQ ID NO: 717 - DNA, 213 bp, Homo Sapiens
caccggtgtggctctttaacaacctttgcttgtcccgataggtcacctttggctcttcagagatgcagggacacacgatgggcttctggttaaccaaactgaattatttgtgccatctctcaatgttgacggacagcctatttttgccaatatcacactgccaggtactgacgttttactttttaaaaagataaggttgttgtggtaagtaca

SEQ ID NO: 718 - DNA, 158 bp, Homo Sapiens
ccgttgggttttctcttccaggggttaattgtgaaattaattttgatgactgtgcaagtaacccttgtatccatggaatctgtatggatggcattaatcgctacagttgtgtctgctcaccaggattcacaggtaaagctccttttactgcaaggccc

SEQ ID NO: 719 - DNA, 135 bp, Homo Sapiens
ttctattcttccttgctttgtgcatgtttatctagactgctgatcttggacttgatattggtgcccagggagaaccccttggatatcgccaggatggtatgtgtctcatatttctcgattaactccagatcaagc

SEQ ID NO: 720 - DNA, 153 bp, Homo Sapiens
aggatggtcttgtgtctgtgttgactgattctcttgtagaccgagattttagatgaagataagcgcttaggcagtgcagtggattactactttattcaagatgacggaagcagatttaaggtaagcccctgactgcgacaagctaaaacccac

SEQ ID NO: 721 - DNA, 157 bp, Homo Sapiens
agttattttcaaacggtctggttttattttagtgctgttcctttgggaaccacggccaaagaagagatggagcggttctggaataagaatataggttcaaaccgtcctctgtctccccacattactatctacaggtaaggaaggattctggagccag

SEQ ID NO: 722 - DNA, 161 bp, Homo Sapiens
aaatggcccttgtcttgcaggtatgacataatgaagacttgctgggatgcagatcccctaaaaagaccaacattcaagcaaattgttcagctaattgagaagcagatttcagagagcaccaatcatgtgagtataccctggccaggcatagaatccccctt

SEQ ID NO: 723 - DNA, 170 bp, Homo Sapiens
tctcccttcctcctttgaacaaacagaacagaacaaacatgacctatgagaaaatgtccagagccctgcgccactactacaaactaaacattatcaggaaggagccaggacaaaggcttttgttcaggtagcacttcctttttctcctttccttcttttgggaggatgct

SEQ ID NO: 724 - DNA, 179 bp, Homo Sapiens
agttaaagttcggttgttttcgtatttcaggtcagcaaattaaaacgtcacattcgctctcatactggagagcgtccgtttcagtgcagtttgtgcagttatgccagcagggacacatacaagctgaaaaggcacatgagaacccattcaggtaggacttctccactccttactgtatt

SEQ ID NO: 725 - DNA, 154 bp, Homo Sapiens
gcaaggagccaggcatttttcttatctcaacatgtgtttgcagcctcctccaaaactgcccagtggagtgttcagtctggaatttcaagattttgtgaataaatggtaagttggctccttgttctctggaagcgtatactctggatttgtcagg

SEQ ID NO: 726 - DNA, 158 bp, Homo Sapiens
tccattggattccttcgcaagggtcaaagactctaaatggaggatctgatgctcaagatggtaatcagccacaacataacggggagagcaatgaagacagcaaagacaaccatgaagccagcacgaagaaaaagtgaggaataggttttaatgggtct

SEQ ID NO: 727 - DNA, 166 bp, Homo Sapiens
ttgtcagctttttgggggtcatttttattcaggatgaagatgcatcagggggcgatcaagatcaggaagaaagaagatggaacaaaaggactcagcagatgcttcatggtcttcaggtattgccgctgttgtctcagaggaaaatgcttcatcaaaggcttttgcc

SEQ ID NO: 728 - DNA, 150 bp, Homo Sapiens
ggtttacgtgcatattttctggcttacgggttttctttatttcctttcagatgcctggaagtcattgacagataaagtccaggaagctcgatcaaatgcccgcctaaagcagctctcatttgcaggtaatggctggaggtgttattccac

SEQ ID NO: 729 - DNA, 150 bp, Homo Sapiens
ggcactttccttctggttcagagcatgtgattgcgaccagcagattgatagctgtacgtatgaagcaatgtataatattcagtcccaggcgccatctatcaccgagagcagcacctttggtaagttgccattctgctactttaaaaatca

SEQ ID NO: 730 - DNA, 150 bp, Homo Sapiens
tggtggtgcatactttatttgtctagaatcgaacagatgtgcagtgccagcaccgatggcagaaagtactaaaccctgagctcatcaagggtccttggaccaaagaagaagatcagagagtaagttctttcttcattggtgtgtgactca

SEQ ID NO: 731 - DNA, 150 bp, Homo Sapiens
aagtggtttcctcagatagagcagtaattgtccatgctctctctaaccaggaaatgttaattttggaggccgtccacaacttccaggttcccatcctgcggtaagtgtcactaggaataccactgaatgagaagctgttgcatatttcac

SEQ ID NO: 732 - DNA, 150 bp, Homo Sapiens
agcgtttcagctccagactctttttgaccaatattgtttcctctttcagaagtgcctagctgccactccatttatatgaggcaagaaggcttcctggctcatcccagcagaacagaagttaagttgtccaccactgaaattccgtgtaaa

SEQ ID NO: 733 - DNA, 208 bp, Homo Sapiens
agcaaccatttttgtgcccatgttttctcattcccttatagggatcgtggaagaataccaattgccatattacaacatggtaccgagtgatccgtcatacgaagatatgcgtgaggttgtgtgtgtcaaacgtttgcggccaattgtgtctaatcggtggaacagtgatgaagtgagtggaactcagtcccctgaagaagtgattcgt

SEQ ID NO: 734 - DNA, 196 bp, Homo Sapiens
tatgtctcctcttccctgcccctgcagactatattgaactccatgcacaaataccagccccggttccacattgtaagagccaatgacatcttgaaactcccttatagtacatttcggacatacttgttccccgaaactgaattcatcgctgtgactgcataccagaatgataaggtaaactcaaggggctttcctt

SEQ ID NO: 735 - DNA, 198 bp, Homo Sapiens
gtcctgctcctgatcctgtttgtattgatttttctaaaaggcttttgtggccacaggaaccaatctgtctctccagttttttccggccagctggcagggagaacagcgacaaacacctagccgagagtatgtcgacttagaaagagaagcaggcaaggtaggaaacatttctttgcaatttaaaatactgtgggttgt

SEQ ID NO: 736 - DNA, 151 bp, Homo Sapiens
cttctccctggctctgactcacccttgttttataacagatgctgcaatgtacaacaactctgaagccctgcccacctctcctatggcacccacaacctatggtatatgtgattcctaattacacaaattaatttgaagggacttactgggg

SEQ ID NO: 737 - DNA, 151 bp, Homo Sapiens
atctcaatcgcctgctctccctttcttctttccagtatggtgactacgaccccagtgttcacaagcggggatttttggcccaagaggaattgcttccaaaaagggtaagagattaaattcccttttcaggaagacatagcagatatgtggt

SEQ ID NO: 738 - DNA, 182 bp, Homo Sapiens
agaccttttcctccctcattcacaggctggcttattagctgtaatggcccagatgggttgttacgtccctgctgaagtgtgcaggctcacaccaattgatagagtgtttactagacttggtgcctcagacagaataatgtcaggtgagttttttgtttcccacttaagttctcattcagtca

SEQ ID NO: 739 - DNA, 150 bp, Homo Sapiens
acatctgggattttgcttcattgtacatatgttttcttccttcagtgaccatgaaagacaccaggttgacagcactggaaactgaagtaccagttgtcgctagaacaggtaagctataaccaggccagtggttagaggaagatgggaggg

SEQ ID NO: 740 - DNA, 150 bp, Homo Sapiens
tcagaccacggtttctatttttcatctagaatgaagatgataaccgagccagtgagagcaagaaacccaaaacggaggacaagaattcagcaggccataagccatccagcaacagagagtacgttcccaaaacatgttgcatgccagtgt

SEQ ID NO: 741 - DNA, 150 bp, Homo Sapiens
atcttctgttacattctgcttcacaggccattctcgaatctccagaaaagcagctaacactaaatgagatctataactggttcacacgaatgtttgcttacttccgacgcaacgcggccacgtggaaggtaagctttctcaggcctgttt

SEQ ID NO: 742 - DNA, 193 bp, Homo Sapiens
ttttcaccccgctccccttagaactggaatgatgaatgggacaatcttatcaaaatggcttccacagacacacccatggcccgaagtggacttcagtacaactcactggaagaaatacacatatttgtcctttgcaacatcctcagaaggccaatcattgtcatttcaggtgagatgcctgcagatcacggat

SEQ ID NO: 743 - DNA, 153 bp, Homo Sapiens
tccttaaggcctctgtgctttttaacaaatggtttcttttgcagttggagttctctccacagacactgtgttgctacggcaaacagttgtgcacaatacctcgtgatgccacttattacagttaccagaacaggtaagcttggccaggtgtgg

SEQ ID NO: 744 - DNA, 198 bp, Homo Sapiens
ggtcatttgctgtgtttgttgacaggtgccaatttgctaattgacagcactggtcagagactaagaattgcagattttggagctgcagccaggttggcatcaaaaggaactggtgcaggagagtttcagggacaattactggggacaattgcatttatggcacctgaggtgagaagcatctttgagtgtgatgacaga

SEQ ID NO: 745 - DNA, 150 bp, Homo Sapiens
ccataatataaagttgttgcgttttgtatttcagaccattgccctcttgaacatttaccgtaaccctcaaaactcttcccagtctgctgacggtttgcgctgtaagttcatacaagttccttccccggttccctgggcttgcgtgtcaga

SEQ ID NO: 746 - DNA, 150 bp, Homo Sapiens
gttctgagttagctgcacatttacctgttggatgttatctgtatttgcagttgtgtactgtcagctatggaaaagtcaagctggtcttgaagcacaacaggtaagagattccatgacaggcctgtcccaaggcactgtcactttctgcgc

SEQ ID NO: 747 - DNA, 165 bp, Homo Sapiens
ttctggccttgttaatggcgtgttctgctttttctttcagtttccccctttctagggtgaggatggttctacacagccacccggagttccttagttgaaaggtgcgccctgctgtgacaggtattctttctttatgtttttctttcatgttaacaatcgaggggg

SEQ ID NO: 748 - DNA, 115 bp, Homo Sapiens
aaatcccttcctctctttctcagataacctgaggaccatggatgctgatgagggtcaagacatgtcccaagtttcaggtgagaccttatgagatagctgtgtgggaagttcatga

SEQ ID NO: 749 - DNA, 130 bp, Homo Sapiens
tacacccctgtcctctctgtcccagggaaattcaactactgaggaggttacggcacaaaaatgtcatccagctggtggatgtgttatacaacgaagagaagcagaaaatatatcctttccggtgttggga

SEQ ID NO: 750 - DNA, 242 bp, Homo Sapiens
agacctcagacaaggcatctcataggaggctttttcataaaactaggctctgctggtagtaaggaggccagtttggaggcaggcgttgagctgtgcacatctccccactccagccaccttctccatatccatcttttatttcatttttccacttggctgagccatccagaaccttttcaatgtataaaatggaatattcttacctcaattcctctgcctacgagtcctgtatggctgggatg

SEQ ID NO: 751 - DNA, 175 bp, Homo Sapiens
actttctctcctgccctcacaagggaaaaagaccttgatgaagttctgcagacccactcagtgtttgtaaatgtttcctaaggtcaggttgccaagaaggaagatctcatcagtgcgtttggaacagatgaccaaactgaaatctgtaagcaggcgggtaacagctgcagcatag

SEQ ID NO: 752 - DNA, 176 bp, Homo Sapiens
cacttcagttatgtacctgatgggtatttctaggcaagaggaggaacgacgtagaagagaggaagagatgatgattcgtcaacgtgagatggaagaacaaatgaggcgccaaagagaggaaagttacagccgaatgggctacatggatccagtaagtcagcctttactgccttcca

SEQ ID NO: 753 - DNA, 178 bp, Homo Sapiens
ttccccattccccattccaaggtaatgtaaatgggaaaaaaagaaaccacacaaagaggatacaggaccctacagaagatgctgaagctgaggacacacccaggaaaagactcaggacggacaagcacagtcttcggaaggtaattgtgttccaggtttgcttgacctgtcagagtgt

SEQ ID NO: 754 - DNA, 167 bp, Homo Sapiens
tgctgaacgcatttggcttatttctccctttcacactttcaaaaatagatcctcgtccctcccaagatgttgtttacacgaggggcttcataacggattctaacggaagacactgaaaaggtaacttgtcagagggggaagagggtggctgcttggggtagggttta

SEQ ID NO: 755 - DNA, 201 bp, Homo Sapiens
tcattgtgtcttccctcctctagctatcttaatgacttggaccgcgtagctgaccctgcctacctgcctacgcaacaagatgtgcttagagttcgagtccccaccacagggatcatcgaatacccctttgacttacaaagtgtcattttcaggtagtaactgagtccatgaaacctatttcccagcttttatgccttgagt

SEQ ID NO: 756 - DNA, 159 bp, Homo Sapiens
tgttgacaatgttttctcccacagggaaaaagcaagcatggttgtccctgaagaaagagaaggcagagatgaaacaaacttagacctagtaagaggcacagcatctgcagatgtttccactgacactcggaaagccggtgagtcctgcactttgtcagg

SEQ ID NO: 757 - DNA, 163 bp, Homo Sapiens
acatttttaatgctcctttctttgacagaaaaagcagacagctctgaaagagaggcactcatgtcagaactcaagatgatgacccagctgggaagccacgagaatattgtgaacctgctgggggcgtgcacactgtcaggtaacccacttccacgaaaatcac

SEQ ID NO: 758 - DNA, 202 bp, Homo Sapiens
agcaaaaggagtgacattcctaatgtgttctttctcccattcttctaggctgacaaacgggctcatcataatgcactggaacgaaaacgtagggaccacatcaaagacagctttcacagtttgcgggactcagtcccatcactccaaggagagaaggtgagtttcctgagaaagctgagtagctggccactactagcttgga

SEQ ID NO: 759 - DNA, 151 bp, Homo Sapiens
tctcatcatttcactgagatatgcatctattacttttacatttcaggccaaaagtgtgatccaagctgtcccaatgggagctgctggggtgcaggagaggagaactgccagaaacgtaagtcagtgaacagcctcagacccatgtgtgacc

SEQ ID NO: 760 - DNA, 195 bp, Homo Sapiens
tgaacttgtcacttcattggtcaatttaatgatttctacaggagcagtttttgcaagaaaggatcaaagtgaacggaaaagctgggaaccttggtggaggggtggtgaccatcgaaaggagcaagagcaagatcaccgtgacatccgaggtgcctttctccaaaaggtacaggagggaagtgtgtgtgtggcctg

SEQ ID NO: 761 - DNA, 196 bp, Homo Sapiens
aggcagcctttataaaagcaaattaacccatgtgggccttaatttttagacagcactaccacctggactggaagtaggactgcaccatacacacctaatttgcctcaccaccaaaacggccatcttcagcaccacccgcctatgccgccccatcccggacattactgtaagctcttgtttttgttgtaagggctat

SEQ ID NO: 762 - DNA, 150 bp, Homo Sapiens
acccattttccttcctggacatgctgcctgcagggccactcatggtgattgtggaattctgcaaatttggaaacctgtccacttacctgaggagcaagagaaatgaatttgtcccctacaaggtatgtcatctcctaatcctgctctggc

SEQ ID NO: 763 - DNA, 181 bp, Homo Sapiens
aaaaatttcccctgcgcttagattcttctactcaaaacaaaagagccaacagaacagaagaaaatgtttcagacggttccccaaatgccggttctgtggagcagacgcccaagaagcctggcctcagaagacgtcaaacgtaaacagctcggtgggttgatcactaaaggagcacgcactg

SEQ ID NO: 764 - DNA, 156 bp, Homo Sapiens
agacatgatgcttcgcttgaaggtaatctttacggttcttctctcaacagctttgaaaagtccagccgcatttcatgagcagagaaggagcttggagcgggccagggtaaggtaccttttttccccctcagaactcccaaagagcattttcagagc

SEQ ID NO: 765 - DNA, 184 bp, Homo Sapiens
tgcacgttgtttgtagctgtagtgcttgattttgggtttctttcacagataaacttctgcactggaggggcctctcctcccctcgttctgcacatggagctctaatccccacgcctgggatgagtgcagaatatgccccgcagggtatttgtaagttgagccttatttcttctacaaatgtcca

SEQ ID NO: 766 - DNA, 175 bp, Homo Sapiens
gtttcccctggatttatgtggtagtagttaactgctgcttctgtttttaggtttcagaagcaggcaacaggaacaagatgtgaactgtttctcttctgcagaaaaagaggctcttcctcctcctcccgcgacggtgggtgtgctgtcctttatcgctgcagtaaaggcgaaggtg

SEQ ID NO: 767 - DNA, 150 bp, Homo Sapiens
acgtgcatgtcctttttcccttttcgtgttctgcaggtggacgttgccataagtcctgtactggccgttgctggggacccacagaaaatcattgccagacttgtaagtgttcatcagtgagagcacacaggtttgatgtggtcaaggaat

SEQ ID NO: 768 - DNA, 150 bp, Homo Sapiens
tgtctctacctcctacatcttatctccaggttggatgattgatgagaacattcgcccaacctttaaagaactagccaatgagttcaccaggatggcccgagacccaccacggtatctggtcataaaggtgagtagggagtaggaggtgct

SEQ ID NO: 769 - DNA, 152 bp, Homo Sapiens
ggttgtttctatttgctaatgctgtttctgttgacttttgacttttctagtttcccagagctatggggacttcccatccggcgttcctggtcttaggctgtcttctcacaggtacggagcccagtcctctctgagttccttgtttgggtgtc

SEQ ID NO: 770 - DNA, 164 bp, Homo Sapiens
agcacttcctgaaataatttcaccttcgtttttttccttctgcaggaggacaccatggaggtggaagagttcttgaaagaagctgcagtcatgaaagagatcaaacaccctaacctggtgcagctccttggtgagtaagcccggggctctgaagagagggtctc

SEQ ID NO: 771 - DNA, 194 bp, Homo Sapiens
atgggcctcactgtctgtttttgctataggtgggaactgcaagatacatggctccagaagtcctagaatccaggatgaatttggagaatgttgagtccttcaagcagaccgatgtctactccatggctctggtgctctgggaaatgacatctcgctgtaatgcagtgggaggtaggtgtggaccagcatcattg

SEQ ID NO: 772 - DNA, 151 bp, Homo Sapiens
gtcctcatggctctgtgactgtgcctcttgtcaggtgtatgagtttagagtcaaagaatctagcatcatagctccagctcccgctgaggatgtggatactcctccaaggaaaaagaagaggaaacaccggtgagtctgtcatgaagctcct

SEQ ID NO: 773 - DNA, 173 bp, Homo Sapiens
cccacctgcattgttcatcatgttaatgccagttcttttttaggtatcatctttatcagaaagtgaggagtcccaggactcatccgacagcataggctcctcacagaaagcccacgggatcctagcacggcgcccatcttacaggtgagtactctcttgtatgaagccctgca

SEQ ID NO: 774 - DNA, 152 bp, Homo Sapiens
ggataactatgttcttccttttcatcatagatattcttactgattctccgggctctgcagctcttgacccggctggtattgtctctacagccaattcctctgaagtcagcaacagcaaaggtgaggtgcgcagggctgccagagaagaggag

SEQ ID NO: 775 - DNA, 154 bp, Homo Sapiens
ctggcacacttcttcacctcctctccttactcttgtttccagatcctgcccctgagctttcatgagctgttgaaccatctggaattcacaggcctgtcatgagagacacgatgagaagtccttaaaggtagatcactgattcacaggggagcag

SEQ ID NO: 776 - DNA, 156 bp, Homo Sapiens
cctcagggatggtagtgacagtcttatttcctattgatacaggatttttttccttgattccttcgtgggactcaagacaggggtgccctgtttactcagcccactgtgctcaacctcttgcaggagtgtgcaggtgagtgagcaagtgcaggatct

SEQ ID NO: 777 - DNA, 158 bp, Homo Sapiens
catccatggaatatgttcttttgcatacagatgccatctcatccggagatgatgaggatgacaccgatggtgcggaagattttgtcagtgagaacagtaacaacaagagtaagtaactgcccggctccgatggtccccgagagaggagcatggaggga

SEQ ID NO: 778 - DNA, 182 bp, Homo Sapiens
ccttgcactcttgtggttgtttttcccattacaggtagagttggctttgtgggacacagctgggcaggaagattatgatcgcctgaggcccctctcctacccagataccgatgttatactgatgtgtttttccatcgacagccctgatagtttaggtgagtggccctgcaccctgatatttg

SEQ ID NO: 779 - DNA, 157 bp, Homo Sapiens
aaggtttccaattcacctttcagctcttcatggaaccagccaggagagagaactggtcagctgctaatcaccaaatgaactccctgatctggcctagggaacagtgggattcacaggcatgggtgacttagaaaaccgggcccagcagaaatgaatc

SEQ ID NO: 780 - DNA, 169 bp, Homo Sapiens
ggtccccatccattcttcctattccctttaggttgttacactctggtaccgagctcccgaagttcttctgcagtccacatatgcaacacctgtggacatgtggagtgttggctgtatctttgcagagatgtttcgtcgaaagtatgggacccacataccctggactacc

SEQ ID NO: 781 - DNA, 150 bp, Homo Sapiens
ccaatctgcttatgaccaggagccactcaagcagcactctcccttcacaggtggtattccaaacacatgactcggagtcaggctgagcaactgctaaagcaagaggtaagtgtggaaccactagcacacagcattctccttgcataagtg

SEQ ID NO: 782 - DNA, 150 bp, Homo Sapiens
ggtgggattttgttgtttgcagctttgactctcccggatcttgcagagcagtttgcccctcctgacattgccccgcctcttcttatcaagctcgtggaagccattgaaaagaaaggtaaccagactgctagagggcatcagttcctttgt

SEQ ID NO: 783 - DNA, 150 bp, Homo Sapiens
tgaccaatttggcttcgtcctcttcctttgcagaaagctgcaggagacacagatgtccaccacctcaaagctggaggaagctgagcataaggttcagagcctacaaacaggtttgatactctccttcctagtaccatggatgtggggagg

SEQ ID NO: 784 - DNA, 150 bp, Homo Sapiens
tcaaagctgcttctgtcatctgtgtgaacatgcgcttttctctctgcagaacctgagagccagaagcaacaaagatgccaaggatccaacgaccaagaactctctggaaagtgagttctgcatgctgaggtctctgtgtgccctcgtcag

SEQ ID NO: 785 - DNA, 150 bp, Homo Sapiens
ggctaatggttctcagagctaagtatcaaggatttcattctcctttgtagggatcctggagcgggttgtgagaaggaatgggcgcgtggatcgtagcctgaaagacgagtgtgatacggtgaaaggatggaggctgtgcaatgggagaat

SEQ ID NO: 786 - DNA, 151 bp, Homo Sapiens
gcctttcaattcactgtcctcactctgacttctcttgtttgttctagaactttgctccccagctgtcttatggctatgatgagaaatcaaccggaggaatttccgtgcctggccccatggtgagccagcagggggagcatggatgacagaa

SEQ ID NO: 787 - DNA, 190 bp, Homo Sapiens
tcagcagggtttttcttgcttgttttcaggctttgtggatttgaccctccatgatcaggtccaccttctagaatgtgcctggctagagatcctgatgattggtctcgtctggcgctccatggagcacccagggaagctactgtttgctcctaacttgctcttggacaggtaagtgacctggctgtagctt

SEQ ID NO: 788 - DNA, 151 bp, Homo Sapiens
ggttttcctctccttccccacagggcgagctactatagaaagggaggctgtgccatgctgccagttaagtggatgcccccagaggccttcatggaaggaatattcacttctaaaacagacacatggtaagtcagccatcatcctccaggta

SEQ ID NO: 789 - DNA, 138 bp, Homo Sapiens
ccatgacactccttccacctcatggcccctttctgttttccagcaagatctttgcaggagtttgccactgtcctcaggaatcttgaagatgaacggatacggatggtgagtagggctgggctactcttggtcccagat

SEQ ID NO: 790 - DNA, 153 bp, Homo Sapiens
tgtaattcctggcttctaggtttctaattctgattttctcctccagaaagatccccagcaggccctcaaggagctggctaagatgtgtatcctggccgactgcacattgatcctcgcctggaggtgagatgagggcttccctgcctcattcag

SEQ ID NO: 791 - DNA, 151 bp, Homo Sapiens
cgtgttcccgtttcctcttgatctcccaggtatttctttgctgtgctggcgatcctcaccatcctcggcgttctcaatgggctggttttgcttcccgtgcttttgtctttctttggaccatatcctgaggtcagtagtgacacggggatgt

SEQ ID NO: 792 - DNA, 178 bp, Homo Sapiens
cctctgtgtatctccttcccaggtaccgcatgcacaagtcccggatgtacagccagtgtgtccgaatgaggcacctctctcaagagtttggatggctccaaatcaccccccaggaattcctgtgcatgaaagcactgctactcttcagcattagtaagtgcctagaagtgcagggaat

SEQ ID NO: 793 - DNA, 172 bp, Homo Sapiens
gctttctttttgctcccccagggcctggtgaaatccccatgggaatgggggctaatccctatggccaagcagcagcatctaaccaactgggttcctggcccgatggcatgttgtccatggaacaagtttctcatggcactcaaaataggtggggtgttattttgtgactctg

SEQ ID NO: 794 - DNA, 150 bp, Homo Sapiens
acttttaccctggatttgcccattcagaacagccaccccatcttttctctcaactgggagtgtgtggtcagtttcctgtggaacacagaggctgcctgtcccattcagacaacgacggatacagaccaggtacgtgtgctttcacctggc

SEQ ID NO: 795 - DNA, 157 bp, Homo Sapiens
ggtggggttttgttaacgtgaatttaatctttttgacagaaataacagcaggctggggaatggagtgctgtatgcctctgtgaacccggagtacttcagcgctgctgatggtaagagtccgggccaccagcactgccagcgtgcagggcaggtagat

SEQ ID NO: 796 - DNA, 157 bp, Homo Sapiens
agtgtaaagttaaccttgctgtgtattttcccttattttaggctgctcctgcgtttggtggatgatttcttgttggtgacacctcacctcacccacgcgaaaaccttcctcaggtgaggcccgtgccgtgtgtctgtggggacctccacagcctgtg

SEQ ID NO: 797 - DNA, 153 bp, Homo Sapiens
gtatcaaggctgccctgactgtcatgctccctgtcttccacagcgggagtcgtgtgaggttggctgtagcagcgcggaaggtgcatatgaagaggaagtactgggtaagaggacacacacgacttttaaaaaataggctgcaccactctagtg

SEQ ID NO: 798 - DNA, 181 bp, Homo Sapiens
ttcaggccaccaacctcattctgttttgttctctatcgtgtccccacagggaaaagcttcactctgaccatcactgtcttcacaaacccaccgcaagtcgccacctaccacagagccatcaaaatcacagtggatgggccccgagaacctcgaagtaagtgcatccacttggggctggtac

SEQ ID NO: 799 - DNA, 156 bp, Homo Sapiens
gtgctgattccctgatgtgccttctacctcttttcttctctcccgccagggagctcgaggacaatatgagtgaccgggttcagtttgtgatcacagcacaggaatgggatcccagctttgaggaggtgagtaccaaagaggcagagaatgggagac

SEQ ID NO: 800 - DNA, 156 bp, Homo Sapiens
accaacatggatggagtggtcactgtgacgcccagaagtatggacgcagaaacctacgtggaaggccagcgcatctcagaaaccaccatgctgcagagtggcatgaaagtgcagtttggggcgtcccatgtatttaagtttgtggaccccagtcag

SEQ ID NO: 801 - DNA, 156 bp, Homo Sapiens
tgcccaccctaatcctgtgtttctttgcctcctatagacatgattcctatggcaatcagttctccacccaaggcaccccttctggcagccccttccccagccagcagactacaatgtatcaacagcaacagcaggtgaggagggtagctgggaatg

SEQ ID NO: 802 - DNA, 154 bp, Homo Sapiens
ctgcctctcttttctccccatacaggacgggctctacgagtgcattctctgtgcctgctgtagcaccagctgccccagctactggtggaacggagacaaatatctggggcctgcagttcttatgcaggtgaggtgctccttaattgctttaaga

SEQ ID NO: 803 - DNA, 184 bp, Homo Sapiens
gaagtcatgggctgcttgtcctgtgctctctccccaggagaaaagccttacagatgctcatgggaagggtgtgagtggcgttttgcaagaagtgatgagttaaccaggcacttccgaaagcacaccggggccaagccttttaaatgctcccactgtgacaggtacgtgcctgaggacaatgctg

SEQ ID NO: 804 - DNA, 150 bp, Homo Sapiens
ccaagctgtgaaggccttttaacagaccaccttccttctgattcccagagaccccaccccctggctacctgagtgaagatggagaaaccagtgaccaccagatgaaccacagcatggacgcaggtcagtcatgcagggtcatgctcttat

SEQ ID NO: 805 - DNA, 150 bp, Homo Sapiens
cctccttctcacgtgtctgtgtttcttttctcctccatgctatggcagtggtgccccgtgctgatgagacaatacttggtgcagccccaggcagtccttttccaggtaatttcctagggacccaaatgatgcccagtgcacactctcctg

SEQ ID NO: 806 - DNA, 204 bp, Homo Sapiens
agcagagtgacccagtgatgtttgtctgttacagatcacggatacacgactctagccaccagtgtgaccctgttaaaagcctcggaagtggaagagattctggatggcaacgatgagaagtacaaggctgtgtccatcagcacagagccccccacctacctcaggtaatgcgttcctggccagggcatctctggggacacctgt

SEQ ID NO: 807 - DNA, 130 bp, Homo Sapiens
tcctctctggatcctcgtgaggtataaagacgagtcctccaccaccagtcaggcacactctaccaccatgaatccactcctgatccttacctttgtggcagctgctcgtgagtatcatgccctgcctcag

SEQ ID NO: 808 - DNA, 150 bp, Homo Sapiens
ggagctgctcctcatcctactcacctttccctcatagtccggaagaccaagggcaaccgaagtacctcacctgtcactgaccccagcatccccattaggaagaaatcaaaggatggcaaaggtatggacagctgggactcaggtgaggtg

SEQ ID NO: 809 - DNA, 150 bp, Homo Sapiens
tgaagtttttgtctgtttctccccctgcagcatctgatgctgttcagatgcagagagagtggagctttgcgcggacacaccctctgctcacctcactgtaccgcagggtgagtggatgtggtattatacctgcttctgagctcgtggcgg

SEQ ID NO: 810 - DNA, 157 bp, Homo Sapiens
actggatctgcttcacacctaggtcccgacatctgtggccctggcaccaagaaggttcatgtcatcttcaactacaagggcaagaacgtgctgatcaacaaggacatccgttgcaaggtgtgcctgggggtggtggcaaatggctgtcatggggaga

SEQ ID NO: 811 - DNA, 157 bp, Homo Sapiens
ctttccctcattccctccccactgcctacttctacttcctcccaggttatgagcagccgttttctgccctacgacaacatcatcacagacgccgtgctcagccttgacgaggacacggtgctttcaacaacagaggtaagaacccatgcctgaggag

SEQ ID NO: 812 - DNA, 151 bp, Homo Sapiens
ttgggcctgtgttatctcctaggttggctctgactgtaccaccatccactacaactacatgtgtaacagttcctgcatgggcggcatgaaccggaggcccatcctcaccatcatcacactggaagactccaggtcaggagccacttgccac

SEQ ID NO: 813 - DNA, 151 bp, Homo Sapiens
cctgacccttctccctatccccagctatgagatcatgcagaagtgctgggaagagaagtttgagattcggccccccttctcccagctggtgctgcttctcgagagactgttgggcgaaggttacaaaaaggtatgttgaggcagggtaggg

SEQ ID NO: 814 - DNA, 185 bp, Homo Sapiens
tccctttctcccctctttgaatgaagagggaaggtgcccacctgtccaccatggctgtgaagatgatccgtgccctgagggatccgaatgtgtgtctgatccctgggaggagaaacacacctgtgtctgtcccagcggcaggtttggtcagtgcccaggtgagagttgaatggttgggtatactt

SEQ ID NO: 815 - DNA, 152 bp, Homo Sapiens
actcaagtccctttcccctctctaccctctcaggactggcagccaccctttgctgtggaagtggacaacttcaggtttaccccccgaatccagaggctgaatgagctagaggtgagaagactaggagctggtggtggggttgggagaatgta

SEQ ID NO: 816 - DNA, 169 bp, Homo Sapiens
tcttcacttcagttgcccctacctattcttgctctcctccgcaggtccagggcttactggagaatggagacagtgtgaccagtcctgagaaggtagccccggaggagggctcaggtaagagaggtaggtctaggtgtggtgtgggtaggctgttgactgcacatcacca

SEQ ID NO: 817 - DNA, 152 bp, Homo Sapiens
ccacactgagcctttttcccttctttgtgtttgcagccacagcacagggtacgagagcgataaccacacaacgcccatcctctgcggagcccaatacagaatacacacgcacggtgtcttcagaggcattcaggtgagcacacagacaggcc

SEQ ID NO: 818 - DNA, 150 bp, Homo Sapiens
catgatgcgctgtgtgtccctgcttctagatgccgacaaaaggatcaaggtggcgaagcccgtggtggagatggatggtgatgagatgacccgtattatctggcagttcatcaaggagaaggtagtgccccctcctgaagtgggtggctc

SEQ ID NO: 819 - DNA, 137 bp, Homo Sapiens
aggaagggcagtgaggattcactggagtctcttcacctctcccaggcatgtcagccacgtggggtgggacccccagaatggatttgacgtgagtaacttcagagtctcttggactccactaaacttccacccaccct

SEQ ID NO: 820 - DNA, 115 bp, Homo Sapiens
caaaaagtgccagccctcacctccctgtcttcttgtctaggttttccgtgtgtatcagggccaacagccagggacctgtatggtaagtctcctaggcctctcccaaccgtgtctc

SEQ ID NO: 821 - DNA, 184 bp, Homo Sapiens
actaagttgccacaggacctgcagcctgcccactctcccctaggtgccgccggatggtggtggttgtctctgatgattacctgcagagcaaggaatgtgacttccagaccaaatttgcactcagcctctctccaggtaagctcaaccctgctctggcaagagaatgagggaatgtgtaggtggg

SEQ ID NO: 822 - DNA, 153 bp, Homo Sapiens
gggctctggggcattaacatatcccattgtgtcctgtttccaggagcctgactacggggccctgtatgagggacgcaaccctggcttctatgtagaggcaaaccctatgccaactttcaaggtacagctcaggcctctgggcataggaagctg

SEQ ID NO: 823 - DNA, 142 bp, Homo Sapiens
cgaagtctcgctcttttcccataggctggagtgcaatggtgtgatctcagctcactgcaacctctgcttcctgggtttaagtgattctcctgcctcagcctcccgagtagctgggattacaggtgactgccaccacgctcag

SEQ ID NO: 824 - DNA, 156 bp, Homo Sapiens
tgttttgttgttcttggcattttctaggagaagcaacagtttcagcgccatctgacccgcccaccaccccagtaccaagacccgacacaaggcagcttcccacagcaggttggacagttcacaggtagggggtgtctgtgtgacgagcagggacag

SEQ ID NO: 825 - DNA, 174 bp, Homo Sapiens
acctgcccagatccttaacctcagcctcttctccagcaggctggagagcacagaagcagagatgcatattccctcagccctagagcctagcacgtccagctccccaaggggcagcacagattcccttaaccaaggtgggtaaaccaatagctaggccattgtcttctgggtacg

SEQ ID NO: 826 - DNA, 119 bp, Homo Sapiens
ctctctccacccaaacccttgtaggatggcagctgtgacccgggatttcggtgagatgcttctgcactctggccgggtcctgccagccgaaggtaagttttcagttccatttcaaagcc

SEQ ID NO: 827 - DNA, 162 bp, Homo Sapiens
tcccctcctcttcttgttctctcattagcttcgcctcaacagcatcaagaagctgtccaccatcgccttggcccttggggttgaaaggacccgaagtgagcttctgcctttccttacaggtaacaaaggggacccctggggcccagatgtggggactcttgg

SEQ ID NO: 828 - DNA, 150 bp, Homo Sapiens
cgacttcagtcttccacttcctatttccacccagttccagcgccaggggcttcagcagacccagcagcagcaacagacagcagctttggtccggcaacttcaacaacagctctctagtaagcctgcctgccttcccaaggagaaccccat

SEQ ID NO: 829 - DNA, 150 bp, Homo Sapiens
tcagcaggaagtgttgaccttttggcctttgtctccttgcaggcaggtgacagcagggacatgtctcgggagatgcaggatgtagacctcgctgaggtgaagcctttggtggagaaaggggaggtgagtggagatcttcctggctacccc

SEQ ID NO: 830 - DNA, 150 bp, Homo Sapiens
gaggccaggcatttttcactagggcctctgctttgcagacagatcttggagctgccctggaaggaggaaactttcttggtgttgcagtcactcctagagcggcaggtgagcaggctgccctggggaagagtggacaaagaagtgctgcag

SEQ ID NO: 831 - DNA, 157 bp, Homo Sapiens
caacacagtctctccctccagcatctggttttgtagcctggatgtgtctgctagtagccgaatggtggtcacaggagacaacgtggggaacgtgatcctgctgaacatggacggcaaagaggtgcgttctccgaggtcctgcctttccctccctcac

SEQ ID NO: 832 - DNA, 155 bp, Homo Sapiens
ttgctgctgcctcgcttatcgtgacctctgttgctctccagatcatcggccgtggcaatgaccaggtggccatcagctccaaatttgagacccgggaggatattggtatgctgccagtggggctggtttctgtgggttccaagaggggaggtgta

SEQ ID NO: 833 - DNA, 162 bp, Homo Sapiens
actgttctgacacaccccacccctctctgcaggtggagtgaccacctttgtggccctctatgactatgagtctaggacggagacagacctgtccttcaagaaaggcgagcggctccagattgtcaacaacacgtgagtgcccccttccctattgcccctcag

SEQ ID NO: 834 - DNA, 169 bp, Homo Sapiens
ctctaaatccctcgccctggctgtgtcctcaggtgctgtgtggccagtcagcagagggacaggaatcattcggccactgttcagacgggagccacacccttctccaatccaagcctggctccagaagagtgagtgtctttacctgacattactgagatctgccgagtgc

SEQ ID NO: 835 - DNA, 156 bp, Homo Sapiens
aacctctacccacccattcctttccagggcactgaagccaaaggcagaagttgatgaggatggagttgtgatgtgctcaggccctgaggagggagaggaggtgggccaggtgaaagggctggggcaagaatggtctggaggtgatggaagggatga

SEQ ID NO: 836 - DNA, 179 bp, Homo Sapiens
tcctctctccccactctcagtctgcagccaggagagcagggacgtcctgtgcgaactgtcagaccaccacaaccacactctggaggaggaatgccaatggggaccctgtctgcaatgcctgtgggctctactacaagcttcacaatgtaagtggactgggatcagcaagaacagggctc

SEQ ID NO: 837 - DNA, 138 bp, Homo Sapiens
aaaaacgggtggttgggcgccgctgtcttttcagtcgggcgctgagtggtttttcggatcatgtctggtggctccgcggattataacaggtatgcagtctgttggcggtcgcggtctgtagtgaaggtcatagggcgc

SEQ ID NO: 838 - DNA, 150 bp, Homo Sapiens
acagacagccgaacagacacggcaggtctcatgagccttcccagccaccgtagtgccggtgccctgagaacaggactgagtgatggcttccaactccagcgatggtgaggctgagtcctgttactatagcaacttcctaggcacactctg

SEQ ID NO: 839 - DNA, 156 bp, Homo Sapiens
ttctttttagtctagtgctccactagctcctctcctactgagctggggtaagaagcggagcgtatacggaggaggcgggatgcatttctgcatcgagcgcacaaaggtgtggcggagggggctccagagctgggaggggtcaatctacgggcgaat

SEQ ID NO: 840 - DNA, 154 bp, Homo Sapiens
taagcccgggacttccttgcctctcttggtagtggtgaatctggagctggcaagacggagaacaccaagaaggtcatccagtatctggcgtacgtggcgtcctcgcacaagagcaagaaggaccaggtgagtgctgcagcccttgtccctgtgg

SEQ ID NO: 841 - DNA, 150 bp, Homo Sapiens
ggggttttgattggctgagggtggagtttgtatctgcaggtttagcgccactctgctggctgaggctgcggagagtgtgcggctccaggtgggctcacgcggtgagtcatatggggaacttctgttgggtgtttggtggttcgaatccca

SEQ ID NO: 842 - DNA, 150 bp, Homo Sapiens
cctagggtgaggcttatgggcttttactcctcagggcaggagacgctgcagagcattacttggacctgctggccctgttgctggatagctcggagccaagggtgggtgtgtcttcaagcttctctgcaatggggtagacgggttggtgtc

SEQ ID NO: 843 - DNA, 151 bp, Homo Sapiens
gggtggccattaacacacaatgggctttctatcctgggcctcagatcgttggtgtctgcactgaagagctacactcagcccagcagtggaacgggcagggcatcctggagctgctgcggacagtgcctatgtgagtacccatgcaaggtgg

SEQ ID NO: 844 - DNA, 334 bp, Homo Sapiens
ctgcgaggaggggagaattcttggggctgagctgggagcccggcaactctagtatttaggataaccttgtgccttggaaatgcaaactcaccgctccaatgcctactgagtagggggagcaaatcgtgccttgtcattttatttggaggtttcctgcctccttcccgaggctacagcagacccccatgagagaaggaggggagcaggcccgtggcaggaggagggctcagggagctgagatcccgacaagcccgccagccccagccgctcctccacgcctgtccttagaaaggggtggaaacatagggacttggggcttggaacctaaggttgt

SEQ ID NO: 845 - DNA, 150 bp, Homo Sapiens
tcccattcccgtgtttccttgcagtgacagcccacacagcgagccaggggccatcgatgaagttgaccatgacaatggcactgagcctcataccagcgatgaaggtgagtgagggggatcctggggacaagggattcttcctggggcctc

SEQ ID NO: 846 - DNA, 129 bp, Homo Sapiens
aggctctgatgtgcttctctctctccctttgcagccgctgtacaaccagccctccgacacccggcagtatcatgagaacatcaaaatgtgagtgctcgcgggcagccgtgcagacacacagaggcaggg

SEQ ID NO: 847 - DNA, 165 bp, Homo Sapiens
gttttctgtctgcctctgccattcccagtgtgaccactcgtgctcagccgtatctcagcaggaggacaggtgccggagcagctcgtgcagctaagcagccaactgcagaaacgtcaggtgggtggtgcattcgcaggcatgctgaagaagcagttccaggcatgg

SEQ ID NO: 848 - DNA, 150 bp, Homo Sapiens
accctcaccctaaatctggcacctgcttctccatctccagagcacaagacgtcccccacccaatgcccggcagctggagaggtctccaacaagcttccaaaatggcctggtgagtgatgcgggatctctctgccctgggtggtggagatg

SEQ ID NO: 849 - DNA, 150 bp, Homo Sapiens
ctgagcctgccctactctgtatctccccgtatagatccgtggccagctgcagtcgcacggcgtgcaagcacgggaggttcggctgatgcggaacaaatcttcaggtgagcttttgttctagtgccctccccttcaagtggccagcctcag

SEQ ID NO: 850 - DNA, 150 bp, Homo Sapiens
cgcgcgtacacacacacacacacacacacacacacacacacacacacacacacgttcttatgtaaccgagcccgggtaaagcagggctgcagaaagcagaaacggcgagcccggctcctgggagcaggtgggacctcctttggcctttgg

SEQ ID NO: 851 - DNA, 199 bp, Homo Sapiens
cctctctccttctgcctcagatgtgaagttcatttccaatccgccctccatggtggcagcggggagcgtggtggccgcagtgcaaggcctgaacctgaggagccccaacaacttcctgtcctactaccgcctcacacgcttcctctccagagtgatcaagtgtgacccggtaagtgagggtgatgtcccaggcagcctt

SEQ ID NO: 852 - DNA, 153 bp, Homo Sapiens
tcgctgttagacatctctctcactgcctgtctctggttctgtcctcaggccacccctgttctccgatgtgtaagggctcccgctgctggggagagagttctgaggattgtcagagccgtgagtctcagggaggcctggagtcagggaagggga

SEQ ID NO: 853 - DNA, 207 bp, Homo Sapiens
tgagaccccttcagaccctacagagaccccactgctctcacagctacaactactgccgggaagacgaggagatctacaaggagttctttgaagtagccaatgatgtcatccccaacctgctgaaggaggcagccagcttgctggaggcgggcgaggagcggccgggggagcaaagccaggtgaaaggctggagctccagcctgtgtc

SEQ ID NO: 854 - DNA, 154 bp, Homo Sapiens
gtgtttccttggggtcatgggggtggcttcatgttagtttttgcaggatccagatgaagaaatggccaaaatcgacaggacggcgagggaccagtgtgggagccaggtaggtccgcccggggttgggcctctgtggaggtccttctccccctgg

SEQ ID NO: 855 - DNA, 118 bp, Homo Sapiens
ctcgctcatccccgaggggcccctgcaacctctccgcgcgaagacggcttcagccctgcagggaaagaaaagtaacttcgcttttctcggaggaaccaggaaggattaagcggcttgg

SEQ ID NO: 856 - DNA, 160 bp, Homo Sapiens
ggcagctccgggtctataaagagaggcgtccgaggacgcgcagggagatttggacgctccggcctgggaggtgcgtcagatccgagctcgccatccagtttcctctccactagtccccccagttggagatctgtaagtagtagttgtcattctgggggca

SEQ ID NO: 857 - DNA, 175 bp, Homo Sapiens
ccctcaccttcccctcttttcccagagctgtcttcccagcccaccatccccatcgtgggcatcattgctggcctggttctccttggagctgtgatcactggagctgtggtcgctgccgtgatgtggaggaggaagagctcaggtggagaaggggtgaagggtggggtctgagatt

SEQ ID NO: 858 - DNA, 154 bp, Homo Sapiens
ctgtccttccctgacctcagcccaacctctactgtgtgcctctgcaggctcggatggcgggtgagcgaggagccagtgctgtcctctttgacatcactgaggatcgagctgctgctgagcaggtacccagggacatttgcgtgttcaaggtggg

SEQ ID NO: 859 - DNA, 185 bp, Homo Sapiens
tggtctctcggcgggaagccgtgcacgcctccagcgttgacactttcccggtgcactttttctggtgggaggggagagcggagcaggctcacgtgtaaccgcgcaggagcctcctctggcttgagccctttcttggtaagtcccaaaccttcccaagacaaccttggccttagcagtagaggagg

SEQ ID NO: 860 - DNA, 150 bp, Homo Sapiens
tgagttaacggctgcctctttctcctggacagggatgggatccccccatacaggatccgtaagcagcaccgcagggagatgcaggagagcgtgcaggtcaatgggcgggtgcccctacctcacattcccgtaagtaccggctttgcggtc

SEQ ID NO: 861 - DNA, 155 bp, Homo Sapiens
cacctggctccactgtgtagctgaggacctgtggctgagcccgctgaccatggaagatcttgtctgctacagcttccaggtggccagagggatggagttcctggcttcccgaaaggtgagcttcccccgaaggcccttcagacgggaaaagggtg

SEQ ID NO: 862 - DNA, 161 bp, Homo Sapiens
cccctgctaatgtctgaggtcccccttctgttcaggagtcatgactctgttctccatcaagagcaaccaccccgggctgctgagtgagaaggctgccagcaagatcaacgagaccatgctgcgcctgggtgagtggccccgggggacttcggtctgaggtc

SEQ ID NO: 863 - DNA, 150 bp, Homo Sapiens
ctggccacactgggtctccctaacacactcctcttctcacccctgcagcccccgcagcctgatgacctctccattgtgtgtttcacaagcggcacgacaggtaagcagaggcacgcagatccccagccatggctacctgcacccttccct

SEQ ID NO: 864 - DNA, 163 bp, Homo Sapiens
cactgtggccttgtttcctgcctgcaggcttggcgggggctccgaggacgccaaggagatcatgcagcatcgcttctttgccggtatcgtgtggcagcacgtgtacgagaagaaggtgcggctgctccccgcatattcacgcgcacgcatgctccccacatat

SEQ ID NO: 865 - DNA, 199 bp, Homo Sapiens
ctcactcctcccctgctcgctgcaggcccgggaccgtggcgcttcgagagattcgtcgttatcagaagtcgaccgagctgctcatccggaagctgcccttccagaggttggtgagggagatcgcgcaggatttcaaaaccgacctgaggtttcagagcgcagccatcggtgcgctgcaggtaagacaaaggcctggagc

SEQ ID NO: 866 - DNA, 197 bp, Homo Sapiens
tagttggcgagtgggctttaggacccaacgggaacccgtgcctcttgcagcagcctaacccagaagcaggggggaatcctgaatcgagctgagagggcttccccggttctcctgggaaccccatcggccccctgccagcacacacctgagcaggtaggaccatgcacaccccttcccaattctttggccgcctttga

SEQ ID NO: 867 - DNA, 170 bp, Homo Sapiens
ctggtttagcgacacgagcaccgcttcttcctcagtaccgcgccggagccttccgcagctgccgcttcagtccgaaggaggaagggaaccaacccactttctcggcgccgcggctcttttctaaaagtgtgagtggccccgggagagggaattgagggggagaaagtggg

SEQ ID NO: 868 - DNA, 150 bp, Homo Sapiens
cctctgctgactctgtctccccaggcagctgcattcagcctcagcggaggacacgcctgtggtgcagttggcagccgagaccccaacagcagagagcaaggtaaggggtgcttgtgtgggtacctgtgctcctggcctggtcgtgtagaa

SEQ ID NO: 869 - DNA, 120 bp, Homo Sapiens
cattggttgcggccatctctgccttgcagacgctccatcctcgggagatgacgaagacggggaggacgaggctgaggacacaggtgtggacacaggtaggagcagggtccagggttcagg

SEQ ID NO: 870 - DNA, 150 bp, Homo Sapiens
ccactgcaacccgactccggagctccgagcatcccttagttttaagtcatggcgggtgcgaacgggtctctgctgcaggcggctccgtgacagctcctgcttcacatgggtagaggagagacggcaaacgtcggggctcccaggacttcg

SEQ ID NO: 871 - DNA, 250 bp, Homo Sapiens
caggagggcggggtaaagccgctttcctctcctttctccctcccccttgtctgcgccacagcccccttctctccccgccccccgggtgtgtcagatttttcagttaataatatcccccgagcttcaaagcgcaggctgtgacagtcatctgtctggacgcgctgggtggatgcggggggctcctgggaactgtgttggagccgagcaagcgctagccaggcgcaagcgcgcacagactgtagccatccga

SEQ ID NO: 872 - DNA, 158 bp, Homo Sapiens
cgcctcttcccaccctagacctggacaaggaggatggacggcccctggagctccgggacctgcttcacttctccagccaagtagcccagggcatggccttcctcgcttccaagaatgtgagtaggaacctggccctggctcatagccacccaggtctg

SEQ ID NO: 873 - DNA, 119 bp, Homo Sapiens
cgtgaccgacatgtggctgtattggtgcagcccgccagggtgtcactggagacagaatggaggtgctgccggactcggaaatggggtaggtgctggagccaccatggccaggcttgctg

SEQ ID NO: 874 - DNA, 151 bp, Homo Sapiens
ctgagacctggggactgatcctcctgcacccctccccagcaccatcgtgaagagtggtctccgtttcgtggcgccagatgccttccatttcactcctcggctcagtcgcctgtgagtgtggccagtgctgggcagtgggagttggggagga

SEQ ID NO: 875 - DNA, 157 bp, Homo Sapiens
agggtttccttctcgctgattccttgtcttggtctccactagggccctggggggaggacgaggagtggacagacaaggcccggcgggtcatcatggagcgtatcggcctcgccactgcagggtaagggccctgtgcctgccctgttctactctctgg

SEQ ID NO: 876 - DNA, 150 bp, Homo Sapiens
aggtgtggtgttgcccaccagcccctcacccgcagtctgtctgcaggatgaagtcgctcacacagtcaccgagagccgggtcctccagaacaccaggcacccgttcctcactgtgagttgccctccccttcccagacagtgtgaggccag

SEQ ID NO: 877 - DNA, 153 bp, Homo Sapiens
tacccactccatttcccaccttctcccctcccaggccatgcacgaggggctgctgatgcccgtggtgaagtcagagggcggcgaggactacacgggagccactgtcatcgagcccctcaaagggtgaggccccaggctgggtgcagtttttac

SEQ ID NO: 878 - DNA, 151 bp, Homo Sapiens
ctgggctggcgtatgacggctgtcgctcctgcatttgcaggtgtctggcctgccaccgtgtctcaaggcggcctgcatacactcgggcatgaccaggaagcaacgggaatctgtcctgcagaaggtgggggcctcatgggcctaggggtga

SEQ ID NO: 879 - DNA, 143 bp, Homo Sapiens
ccgctcagtgtctctctcttgctctcgctctcgctctccccctctttctctctttctctctttttccgcgaggcctacacgacgccaggggtttgggtgcgtgttggggagggggagggggagcccatggggctccggagact

SEQ ID NO: 880 - DNA, 224 bp, Homo Sapiens
caggaagcctgtgttccgtacgacaatatggcggcgcttagttgcatgaaggcggaaactctgtgacttccggtccgtagtggggcctgcggtgggagtgggaaggaaggcggagggaaccatgcgaggttctgagaattgcggcgagggtcgcctcgagagacggtttctgaggtgggggccggacggtgcggggatcagaggcgggggcggggatatagagg

SEQ ID NO: 881 - DNA, 214 bp, Homo Sapiens
gaacttgccggttaagcaggcccccgtgtctctccctgttcccctgcagaaggccgggagtgtgtcaactgtggggccacagccacccctctctggcggcgggacggcaccggccactacctgtgcaatgcctgtggcctctaccacaagatgaatgggcagaaccgaccactcatcaagcccaagcgaagactggtaggagcgggcacaggtg

SEQ ID NO: 882 - DNA, 220 bp, Homo Sapiens
gtatcaacgctctgtgggtcgtgtgcgtgcgaggggggcgacgtaagggcgctccgcgagcccgtctctcctcgaatgaaaggaaacaacctccggcgacagagccccgctctcaggcactgctggagaaccgagaccgacttctttctctttaccctcattggcgcttctctcctgcagtccgcctctgggccctgccggtgagtccccacggaaccct

SEQ ID NO: 883 - DNA, 158 bp, Homo Sapiens
tgcttctcttccttctcccccaggagactgaggcatgccctgtggccctcacttccagacctgcaccgggtcctaggccagtaccttagggacactgcagccctgagcccggtgagtgtgcttccctcccctgtgcccaccaccaaccctgcctggta

SEQ ID NO: 884 - DNA, 297 bp, Homo Sapiens
ctttgtgtgccccgctccagcagcctcccgcgacgatgcccctcaacgttagcttcaccaacaggaactatgacctcgactacgactcggtgcagccgtatttctactgcgacgaggaggagaacttctaccagcagcagcagcagagcgagctgcagcccccggcgcccagcgaggatatctggaagaaattcgagctgctgcccaccccgcccctgtcccctagccgccgctccgggctctgctcgccctcctacgttgcggtcacacccttctcccttcggggagacaacgacg

SEQ ID NO: 885 - DNA, 151 bp, Homo Sapiens
aggcctcttgtttcctccccaggcccctgagcctctgagctccttgaagtccatggcggaacgggcagccatcagctctggcattgaggaccctgtgccaacgctgcacctgaccgagcgaggtgagggacccaggatggtggggaagcag

SEQ ID NO: 886 - DNA, 166 bp, Homo Sapiens
ctatgggtgcccttctccacagatcatccagctgaccccggtgcctgtgagcacacccagcggcctggtgccgcccctgagcccagccacactccctggacccacctctcagcctcagaaggtcctgttgccctcctccaccaggtaattgcagctgagcccatac

SEQ ID NO: 887 - DNA, 151 bp, Homo Sapiens
gaggacctgtgggactctgcactgaggccctctctcccctccagggccgcctgcctgtgaagtggatggcgcccgaggccttgtttgaccgggtgtacacacaccagagtgacgtgtgagtcctgccggcggtcactgtcctaccccacaa

SEQ ID NO: 888 - DNA, 154 bp, Homo Sapiens
gggtgagactgacctctcttctcctgcccctgcctaggcccgcgatgctcccagcccggtgagacctgcctgaatggcgggaagtgtgaagcggccaatggcacggaggcctgcgtgtgagtaccacccctgcgggacctgttgctttgtcgag

SEQ ID NO: 889 - DNA, 343 bp, Homo Sapiens
ctgcagttcgcttgtgcccggcagcccgagctcgccatgatgcattgctcttactgggaccacgacagcaagaccggcgcgctgcattcgcgcctcgatctctgagagcccaccgcatgccggtgcagacggatgcgaggatgcagggacgcgcgacgccggccccggtcgcagccgacgacgccgccgccagcctgacctcacaccctctgggcccgcctctggagccagcgcccagggtccctctgtgctttttcgctttcctaagctcctgtcgctcctctttgtcccctcagtttatgtcctcctgtgctcacctccctgacctctgtgaccttgcact

SEQ ID NO: 890 - DNA, 199 bp, Homo Sapiens
cacccaccgctgtgttgcagctacctgaccgacgttgaccgcatcgccaccttgggctacctgcccacccagcaggacgtgctgcgggtccgcgtgcccaccaccggcatcatcgagtaccctttcgacctggagaacatcatcttccggtaccgcccgggccacagcaggcggggagggggcactgagaggctcattt

SEQ ID NO: 891 - DNA, 127 bp, Homo Sapiens
aggaagggagcctcaaaggccaaggccagccaggacaccccctgggatcacactgagcttgccacatccccaaggcggccgaaccctccgcaaccaccagcccaggtcagtctcagcccccagagag

SEQ ID NO: 892 - DNA, 206 bp, Homo Sapiens
gactctcctgtctccgctccctgccttgctcgcaggcagccacctggcgagtctgacatggctgtcagcgacgcgctgctcccatctttctccacgttcgcgtctggcccggcgggaagggagaagacactgcgtcaagcaggtgccccgaataacgtgagtatcgctccgggccgccgggaacgcccggtgggttttcgtgggtg

SEQ ID NO: 893 - DNA, 166 bp, Homo Sapiens
cctcctctgcgttcgacgcagcctccgcccggcctcccaggatgcagcgcgctggcgggaggtttggagcagatggataccgtatcgacgtggggcctccggtatgttgccgctgcgttgaggtaggatggggctggcgagtcttcccttcccaggacttcgcaga

SEQ ID NO: 894 - DNA, 169 bp, Homo Sapiens
actacatttcccaggaggcagcgggtctacgccgtcgccgtcgtcggagagcggagacgctgggcgcgctgtggggcgggggcgaggttcgggctggttgttccgttgcgagctgcagctgcgatctctgtggtaggcccaggtgagtgagcgcctctgatggaagtta

SEQ ID NO: 895 - DNA, 155 bp, Homo Sapiens
ccgtccgcgctacatactgcgcctgcgcaagggctgtggcccttttcccaccccctagcgccgctgggcctgcaggtctctgtcgagcagcggacgccggtctctgttccgcaggatggtgagtggatgcctcggtctcggggctttagatgcat

SEQ ID NO: 896 - DNA, 162 bp, Homo Sapiens
cagtggctcaggaaaccaaggggcccacacaggaaggagccgagtgggactttcctctcgctgcctcccggctctgcccgcccttcgaaagtccagggtccctgcccgctaggtaagagctggcgatgccgcagggctcggcccagacactgggggaggatg

SEQ ID NO: 897 - DNA, 153 bp, Homo Sapiens
gctgatcctccaccttccttcacccccacacagcccccccttgcctggacggaagcccgtgtgcaaatggaggtcgttgcacccagctgccctcccgggaggctgcctgcctgtgagtgcctggctcagagccaccagtgggccctgtgtgtg

SEQ ID NO: 898 - DNA, 220 bp, Homo Sapiens
gaacatggtgcgcaggttcttggtgaccctccggattcggcgcgcgtgcggcccgccgcgagtgagggttttcgtggttcacatcccgcggctcacgggggagtgggcagcgccaggggcgcccgccgctgtggccctcgtgctgatgctactgaggagccagcgtctagggcagcagccgcttcctagaagaccaggtaggaaaggccctcgaaaagtc

SEQ ID NO: 899 - DNA, 148 bp, Homo Sapiens
gtgtgttgggggatagcctcggtgtcagccatctttcaattgtgttcgcagccgccgccgcgccgccgtcgctctccaacgccagcgccgcctctcgctcgccgagctccagccgaaggagaaggggggtaagtttccccgtctgccc

SEQ ID NO: 900 - DNA, 193 bp, Homo Sapiens
cacgtctgcccctctctcccctgcggccagccctctacagccacaagcccgaggtggcccagtacacccacacgggcctgctcccgcagactatgctcatcaccgacaccaccaacctgagcgccctggccagcctcacgcccaccaagcaggtaaggtccaggcctgctggccctcccttggcctgtgacag

SEQ ID NO: 901 - DNA, 240 bp, Homo Sapiens
ggcagaagagaggcagacagactgacagacacgtagaccaacagtgcggccccagggttcgtccccagactcgctcgctcatttgttggcgactggggctcagcgcagcgaagcccgatgtggtccggaggcagtgggaaggcgcggggctgggaggccgcggcgggagggaggagcagccccggcaggctcaggtgaaacccccaccctgtccctcagccccctcctcctaaagacctg

SEQ ID NO: 902 - DNA, 348 bp, Homo Sapiens
tattaccggcagaaccagcagcgctggcagaactccatccgccactcgctgtccttcaatgactgcttcgtcaaggtggcacgctccccggacaagccgggcaagggctcctactggacgctgcacccggactccggcaacatgttcgagaacggctgctacttgcgccgccagaagcgcttcaagtgcgagaagcagccgggggccggcggcgggggcgggagcggaagcgggggcagcggcgccaagggcggccctgagagccgcaaggacccctctggcgcctctaaccccagcgccgactcgcccctccatcggggtgtgcacgggaagaccggccagctagag

SEQ ID NO: 903 - DNA, 198 bp, Homo Sapiens
cacccggttccatctacctttcccccaccccaggtctcctcttggctctgccaggagccggagccctgccaccctggctttgacgccgagagctacacgttcacggtgccccggcgccacctggagagaggccgcgtcctgggcagaggtgagggcgcgctgccggtgtccctgggcggagtagggaggggttggaaa

SEQ ID NO: 904 - DNA, 259 bp, Homo Sapiens
cgatgagggtctggccagcgccgcggcgcggggactagtggagaaggtgcgacagctcctggaagccggcgcggatcccaacggagtcaaccgtttcgggaggcgcgcgatccaggtagctggggccccagggcctcgccggcagggggcgcgcgaacgcggggcgcggcctcggcggatcggggctggaacctagatcgccgatgtagatttgtacaggagtctccgttggccggaggtgtgcattccacgcgtaaaa

SEQ ID NO: 905 - DNA, 150 bp, Homo Sapiens
cgctgctgccttgatgggctccgcggcccgagcgcctcttttcgggattaaaagcgccgccagctcccgccgccgccgccgtcgccagcagcgccgctgcagccgccgccgccggagaagcaaccgcgtaagtggcaacttttccctctt

SEQ ID NO: 906 - DNA, 150 bp, Homo Sapiens
actcactgaccctctcccttgacacagggcagccgctctggctctagctccagctccgggaccctctgggaccccccgggacccatgtgacccagcggcccctcgcgctgtaagtctcccgggacggcagggcagtgagggaggcgaggg

SEQ ID NO: 907 - DNA, 198 bp, Homo Sapiens
agcgaggacatctggaagaaattcgagctggtgccatcgccccccacgtcgccgccctggggcttgggtcccggcgcaggggacccggcccccgggattggtcccccggagccgtggcccggagggtgcaccggagacgaagcggaatcccggggccactcgaaaggctggggcaggaactacgcctccatcatacgc

SEQ ID NO: 908 - DNA, 152 bp, Homo Sapiens
caagaggccaatgagggggcagtgcccggcattatgcaacccgcctccccgcccgcccggtggagcttccactcggctgcgggctggagcggcggcgggcaggcgtgcggaggacactcctgcgaccaggtaggcatctctgcggccatcct

SEQ ID NO: 909 - DNA, 163 bp, Homo Sapiens
ctacctgtaactgggcctgttgctgtctcctagcacaaactctcagagcccatccccacccagcagttccattgcctacagcctcctgagtgccagctcagagcaggacaacccgtccaccagtggctgcaggtacgtcgggtgaggctggaggagaggtctg

SEQ ID NO: 910 - DNA, 296 bp, Homo Sapiens
gatggcgcctcagaagcacggcggtgggggagggggcggctcggggcccagcgcggggtccgggggaggcggcttcgggggttcggcggcggtggcggcggcgacggcttcgggcggcaaatccggcggcgggagctgtggagggggtggcagttactcggcctcctcctcctcctccgcggcggcagcggcgggggctgcggtgttaccggtgaagaagccgaaaatggagcacgtccaggctgaccacgagcttttcctccaggcctttgagagtgagtgtgtgcgaggctttg

SEQ ID NO: 911 - DNA, 283 bp, Homo Sapiens
gggctccgtagacgctttccgcatcactctccttcctcgggctgccgggagtcccgggacctggcggggccggcatgacgggcttctcgggggcccgccgcacgcccggcagcctccggagacgcgcgccgagcccggctcccacggcctctgaggctcggcggggctgcggctgcctggcgggcgggctccggagctttcctgagcggcattagcccacggcttggcccggacgcgaccaaaggctcttctggagaagcccagagcactgggcaatcgttac

SEQ ID NO: 912 - DNA, 162 bp, Homo Sapiens
ctgccttctcccctgaagagagacgcggggggaggggggtgcggcgagcggccccgctctctccccaccgctccgctcgcaccccagtgtaatgagggtcaccccctccccccagctggcccgggagggggcgcggggcacggtaactagtgcgctggggtg

SEQ ID NO: 913 - DNA, 10 bp, Artificial Sequence
  synthetic sequence
cctcagcaag

SEQ ID NO: 914 - DNA, 10 bp, Artificial Sequence
  synthetic sequence
cttgctgagg

SEQ ID NO: 915 - DNA, 27 bp, Artificial Sequence
  synthetic sequence
  misc_feature (6)..(17): n is a, c, g, or t
cccaannnnnnnnnnnncctcagcaag

SEQ ID NO: 916 - DNA, 34 bp, Artificial Sequence
  synthetic sequence
gtgactggagttcagacgtgtgctcttgctgagg

SEQ ID NO: 917 - DNA, 13 bp, Artificial Sequence
  synthetic sequence
  modified_base (13)..(13): dideoxy cytidine, or ddC
cgaccctcagccc

SEQ ID NO: 918 - DNA, 29 bp, Artificial Sequence
  synthetic sequence
  modified_base (1)..(1): phosphate group
  misc_feature (25)..(26): PTO bond between two adjacent bases
  misc_feature (26)..(27): PTO bond between two adjacent bases
  misc_feature (27)..(28): PTO bond between two adjacent bases
  misc_feature (28)..(29): PTO bond between two adjacent bases
ggctgagggtcgtgtagggaaagagtgta

SEQ ID NO: 919 - DNA, 51 bp, Artificial Sequence
  synthetic sequence
aatgatacggcgaccaccgagatctacactctttccctacacgacgctctt

SEQ ID NO: 920 - DNA, 52 bp, Artificial Sequence
  synthetic sequence
  misc_feature (25)..(31): n is a, c, g, or t
caagcagaagacggcatacgagatnnnnnnngtgactggagttcagacgtgt